European Patent Application EP 4 567 118 A2, published June 11, 2025. Title: TRANSGENIC MAMMALS AND METHODS OF USE THEREOF. Applicant: Trianni, Inc. Application EP. The sequence listing filed with the application follows.

SEQUENCE LISTING (295 sequences)

SEQ ID NO: 1 - DNA, 300 bp, Bos taurus
  source 1..300: mol_type = genomic DNA
caggtgcagctgcgggagtcgggccccagcctggtgaagccgtcacagaccctctccctcacctgcacggtctctggattctcattgagcgacaaggctgtaggctgggtccgccaggctccagggaaggcgctggagtggctcggtggtatagacactggtggaagcacaggctataacccaggcctgaaatcccggctcagcatcaccaaggacaactccaagagccaagtctctctgtcagtgagcagcgtgacaactgaggactcggccacatactactgtactactgtgcaccag

SEQ ID NO: 2 - DNA, 293 bp, Bos taurus
  source 1..293: mol_type = genomic DNA
caggtgcagctgcgggagtcgggccccagcctggtgaagccctcacagaccctctccctcacctgcacggtctctggattctcattgagcagctatggtgtaggctgggtccgccaggctccagggaaggcgctggagtgtcttggtggtataagtagtggtggaagcacaggctataacccagccctgaaataccggctcagcatcaccaaggacaactccaagagccaagtctctctgtcactgagcagcgtgacaactgaggacacggccacatactactgtgcgaagga

SEQ ID NO: 3 - DNA, 293 bp, Bos taurus
  source 1..293: mol_type = genomic DNA
caggtgcagctgcgggagtcgggccccagcctggtgaagccctcacagaccctgtccctcacctgcacggtctctggattctcattaagcgataatagtgtaggctgggtccgccaggctccaggaaaggcgctggagtggctcggtgtcatatatagtggtggaagcacaggctataacccagccctgaaatcccggctcagcatcaccaaggacaactccaagagccaagtctctctatcactgagcagcgtgacaactgaggacacggccacatactactgtgcaagaga

SEQ ID NO: 4 - DNA, 293 bp, Bos taurus
  source 1..293: mol_type = genomic DNA
caggtgcagctgcgcgagtcgggccccagcctggtgaagccctcacagaccctctccctcacctgcacggtctctggattctcattgagcagctatgctgtaagctgggtccgccaggctccagggaaggctctggagtggcttggtgatataagcagtggtggaagcacaggctataacccagccctgaaatcccggctcagcatcaccaaggacaactccaagagccaagtctctctgtcagtgagcagcgtgacacctgaggacacggccacatactactgtgcgaagga

SEQ ID NO: 5 - DNA, 293 bp, Bos taurus
  source 1..293: mol_type = genomic DNA
caggtgcagctgcgggagtcgggccccagcctggtgaagccctcacagaccctctccctcacctgcacggtctctggattctcactgagcagctatgctgtaggctgggtccgccaggctccagggaaggcgctggagtggctcggtggtataagcagtggtggaagcacatactataacccagccctgaaatcccggctcagcatcaccaaggacaactccaagagccaagtctctctgtcagtgagcagcgtgacacctgaggacacggccacatactactgtgcgaagga

SEQ ID NO: 6 - DNA, 293 bp, Bos taurus
  source 1..293: mol_type = genomic DNA
caggtgcagctgcgggagtcgggccccagcctggtgaagccctcacagaccctctccctcacctgcacgatctctggattctcattgagcagctatgctgtaggctgggtccgccaggctccggggaaggcgctggagtgggttggtggtataagtagtggtggaagcacatgccttaacccagccctgaaatcccggctcagcatcaccaaggacaactccaagagccaagtctctctgtcagtgagcagcgtgacaactgaggacacggccacatactactgtgcgaagga

SEQ ID NO: 7 - DNA, 293 bp, Bos taurus
  source 1..293: mol_type = genomic DNA
caggtgcagctgcaggagtcgggccccagcctggtaaagacctcacagaccctctccctcacctgcacggcctctggattatcattaaccagatatggtatacactgggtccgccaggctccaggaaaggcgctggagtggcttggtgatataagcagtggtggaagcacaggctataacccaggcctgaaatcccggctcagcatcaccaaggacaactccaagagccaagtctctctgtcactgagcagcctgacacctgaggactcagccacatactactgtgcaagaga

SEQ ID NO: 8 - DNA, 293 bp, Bos taurus
  source 1..293: mol_type = genomic DNA
caggtgcagctgcgggagtcgggccccagcctggtgaagccctcacagaccctctccctcacctgcacggtctctggattctcattgagcagcaatggtgtaggctgggtccgccaggctccagggaaggcgctggagtgggttggtggtatagataatgatggagacacatactataacccagccctgaaatcccggctcagcatcaccaaggacaactccaagagccaagtctctctgtcagtgagcagcgtgacacctgaggacacggccacatactactgtgcaaaaga

SEQ ID NO: 9 - DNA, 293 bp, Bos taurus
  source 1..293: mol_type = genomic DNA
caggtgcagctgcgggagtcgggccccagcctggtgaagccctcacagaccctctccctcacctgcacggtctctggattctcattgagcagcaatggtgtagtctgggtccgccaggctccagggaaggcgctggagtggctcggtggtatatgcagtggtggaagcacaagctttaacccagccctgaaatcccggctcagcatcaccaaggacaactccaagagccaagtctctctgtcagtgagcagcgtgacacctgaggacacggccacatactactgtgcaagaga

SEQ ID NO: 10 - DNA, 293 bp, Bos taurus
  source 1..293: mol_type = genomic DNA
caggtgcagctgcaggagtcgggccccagcctggtgaagccctcacagaccctgtccctcacctgcacggtctctggattctcattaagcgacaatgctgtaggctgggtccgccaggctccaggaaaggcgctggagtagcttggtggtatagataatgatggatacacaaggtataacccagccctgaaatcccggctcagcattaccaaggacaactccaagagctaagtctctgtgtcagtgagcagcgtgacaactgaggactcggccgtgtactactgtgcgaagga

SEQ ID NO: 11 - DNA, 293 bp, Bos taurus; identical to SEQ ID NO: 6
  source 1..293: mol_type = genomic DNA

SEQ ID NO: 12 - DNA, 293 bp, Bos taurus
  source 1..293: mol_type = genomic DNA
caggtgcagctgcaggagtcgggccccagcctggtgaagacctcacagacactctccctcacttgcacggcctctggattatcattaaccagatatggtatacactgggtccgccaggctccaggaaaggcgctggagtggcttggtgatataagcagtggtggaagcacaggctataacccaggcctgaaatcccggctcagcatcaccaaggacaactccaagagccaagtctctctgtcactgagcagcctgacgcctgaggactcagccacatactactgtgcaagaga

SEQ ID NO: 13 - DNA, 293 bp, Bos taurus
  source 1..293: mol_type = genomic DNA
aaggtgcagctgcaggagtcgggtcccagcctggtgaagccctcacagaccctctccctcacctgcacgacctctggattctcattgaccagctatggtgtaagctgggtccgccaggctccagggaaggcgctggagtggctcggtggtatagatagtggtggaagcacaggctataacccaggcctgaaatccaggctcagcatcaccagggacaactccaagagccaagtctctctgtcagtgagcagcgtgacacctgaggacacggccacatactactgtgcgaagga

SEQ ID NO: 14 - DNA, 288 bp, Bos taurus
  source 1..288: mol_type = genomic DNA
gaggtgcagctgcgggagtggggccccagcctggtgaagccctcacagaccctctccctcaccttcatggtctctggattctcattgaccagctatggtgtagattgggtccgccaggctccagggaaggtgccggaatgggttggtggtataagcagtggtggaagtacatactataacccagccctgaaattcccggctcagcatcacgagggaaacctccaagagccaagtctctctgagcagcgtgacaactgaggacacggccgtgcactactgtgtgaagga

SEQ ID NO: 15 - DNA, 288 bp, Bos taurus
  source 1..288: mol_type = genomic DNA
aaggtgcagctgcgggagtggggccccagcctggtgaagccctcacagaccctctccctcaccttcatggtctctggattctcattgaccagctatggtgtagattgggtccgccaggctccagggaaggtgccggaatgggttggtggtataagcagtggtggaagtacatactataacccagccctgaaattcctggctcagcatcacgagggaaacctccaagagccaagtctctctgagcagcgtgacaactgaggacacggccgtgcactactgtgtgaagga

SEQ ID NO: 16 - DNA, 285 bp, Bos taurus
  source 1..285: mol_type = genomic DNA
aaggtgcagctgcaggagtcgggtcccagcctggtgaagccctcacagaccctctccctcacctgcacggtctctggattctcattgagcagctatggtatacactgggtccgccaggctccaggaaaggcgctggagtggcttggtgatataagcagtggtggaagcacaggctataacccaggcctgaaatcccggctcagcatcaccaaggacaactccaagagccaagtctctctgtcactgagcagcctgacgcctgaggacacagccacatactactgt

SEQ ID NO: 17 - DNA, 311 bp, Bos taurus
  source 1..311: mol_type = genomic DNA
ccgatgcagctgcaggagtcaggccccagcctggtgaagccctcacagaccctttccttcacctgcactgtgtctggattctcattaaccaacaatggtgtaggctgggtccgccaggctccacaaaagggattggagttggttggtatcatatgtacaatatgatatatatatgatatggaagcacatactaccacccagcccttaagtccaggctcagcatcaccagcgacatctccaagagcctagtctcttgtattactgagcagcgtgacaactgaggacacggccctgtagtactgtgcaaaaga

SEQ ID NO: 18 - DNA, 287 bp, Bos taurus
  source 1..287: mol_type = genomic DNA
cagatgagctgcagcagtcgggccagaactggtgaaccctcactcaccctctcctgacgtgcactgtctcttcttactccatcacgtggttattgtcggaactggattcgccaggccctagggaaggggctagagcagatgtcataaataagctatgatggtgacacttactacagcccctgcatcaagatcacacctccatctgcagagacatccaagaatcagttctctctgcagctgagctctgtgaccactgaggacacggcagtgtgctgctgtgcaagaga

SEQ ID NO: 19 - DNA, 294 bp, Bos taurus
  source 1..294: mol_type = genomic DNA
caggtgaaggtgcaggagtcgggcccagacctggtgaagccctcgcagatcgtctccctcacatgtgctgtctctggttactccatcacgtggttatggtgagagctgggtccaccaggccccagcgaaggggctagagtggatgggaagcatatattataatggtgacacttaccacagcccctccatcaagagccacacctccatctccaggggcacgtctaagaaccagtcctccctgcagctgagctccgtgaccactgtggacacagctgtgtattactgtgcaagaga

SEQ ID NO: 20 - DNA, 155 bp, Bos taurus
  source 1..155: mol_type = genomic DNA
ccagtgcagctgcaggagcagggtccagaactgcggaagctctcacctgtgccatctctggttgctccatcaccaatggttactggtaaccagtactccctgcagctaagctctgtgacaaccaaggacacggcagtatgctgctgtgcaagaga

SEQ ID NO: 21 - DNA, 271 bp, Bos taurus
  source 1..271: mol_type = genomic DNA
ccagatgcactgcagcagtcgggcccagaactagtgagccctcactgaccctctcctcacgtgcactatctctggttactccatcaagtggttattgagggaactggttttgccaggccccagggaaggggctagagcagatggcatgcataaactaagatggtgacacttactacatcccctccatcaagagccacacctccaatcagttctccctgcagctgaactctgtgaccattgaggacacggccatgtgttgctgggcaagaga

SEQ ID NO: 22 - DNA, 296 bp, Bos taurus
  source 1..296: mol_type = genomic DNA
caggtgaaggtgcaggagtcgggcccagagacctggtgaagccctcgcagatcgtctccctcacatgtgctgtctctggttactccatcacgtggttatggtgggagctggatccaccaggccccagcgaaggggctagagtagatgggaagcatatattataatggtgacacttaccacagcccctccttcaagagccacacgtccatctccaggggcacgtctaagaaccagtcctccctgcagctgagctccgtgaccactgtggacacagctgtgtgttactgtgcaagaga

SEQ ID NO: 23 - DNA, 155 bp, Bos taurus
  source 1..155: mol_type = genomic DNA
ccagtgcagctgcaggagcagggtccagaactgcggaagctctcacctgtgccatctctggttgctccatcaccagtggttactggtaaccagtactccctgcagctaagctctgtgacaaccaaggacacggcagtatgctgctgtgcaagaga

SEQ ID NO: 24 - DNA, 155 bp, Bos taurus
  source 1..155: mol_type = genomic DNA
ccagtgcagctgcaggagcagggtccagaactgcggaagctctcacctgtgccatctctggttgctccatcaccagtggttactggtaaccagtactccctgcagctaagctctgtgatgaccaaggacacggcagtatgctgctgtgcaagaga

SEQ ID NO: 25 - DNA, 291 bp, Bos taurus
  source 1..291: mol_type = genomic DNA
cccagatgcactgctgcagtcgggccagaactggtgaagccctcactgactgtctcctcacttgcactgtctctgcttactccatcacgtggttattgtgggaactggattcgccaggccccagggaaggggctagagcagatgacatgcataaactatgatggtgacacttactacagcccctccatcaagagccacatctccatctgcagggacatccaagaatcagttctccctgcagctgagctctgtgaccactgaggacacggccatgtgttgctgtgcaagaga

SEQ ID NO: 26 - DNA, 294 bp, Bos taurus
  source 1..294: mol_type = genomic DNA
caggtgaaggtgcaggagtcgggcccagaactggtgaagccctcgcagatcgtctccctcacatgtgctgtctctggttactccatcacgtggttatggtgggagctggatccaccaggcccgagggaaggggctagagtagatgggaagcatatattataatggtgacacttaccacagcccctccatcaagagccacacgtccatctccaggggcacgtctaagaaccagtcctccctgcagctgagctctgtgaccactgaggacacagctgtgtattactgtgcaagaga

SEQ ID NO: 27 - DNA, 155 bp, Bos taurus
  source 1..155: mol_type = genomic DNA
ccagtgcagctgcaggagcagggtccagaactgcggaagctctcacctgtgccatctctggttgctccatcaccagtggttactggtaaccagtactccctgcagctaagctctgtgacgaccaaggacacggcagtatactgctgtgcaagaga

SEQ ID NO: 28 - DNA, 155 bp, Bos taurus
  source 1..155: mol_type = genomic DNA
ccagtgcagctgcaggagcagggtccagaactgcggaagctctcacctgtgccatctctggttgctccatcaccagtggttactggtaaccagtactccctgcagctaagctctgtgatgaccaaggacacggcagtatactgctgtgcaagaga

SEQ ID NO: 29 - DNA, 292 bp, Bos taurus
  source 1..292: mol_type = genomic DNA
caggtgaaggtgcaggagtcgggcccagaactggtgaagccctcgcagatcatctccctcacatgtgctgtctctggttactccatcacgtggttatggtgggagctggatccaccaggccccagggaaggggttagagtggatgggaagcatatattataatggtgacacttaccacagcccctccatcaagagccacacctccatctgcagagacatccaacaatcagttctccctgtagctgagctctgtgaccactgaggacacagctctgtgttgctgtgcaagaga

SEQ ID NO: 30 - DNA, 291 bp, Bos taurus; identical to SEQ ID NO: 25
  source 1..291: mol_type = genomic DNA

SEQ ID NO: 31 - DNA, 294 bp, Bos taurus
  source 1..294: mol_type = genomic DNA
caggtgaaggtgcaggagtcgggcccagaactggtgaagccctcgcagatcgtctccctcacatgtgctgtctctggttactccatcacgtggttatggtgggagctggatccaccaggccccagggaaggggctagagtggatgggaagcatatattataaaggtgacacttaccacagcccttccatcaagagccacacgtccatctccaggggcacgtctaagaaccagtcctccctgcagctgagctctgtgaccactgaggacacagctgtgtattactgtgcaagaga

SEQ ID NO: 32 - DNA, 171 bp, Bos taurus
  source 1..171: mol_type = genomic DNA
ccagtgcagctgcaggagtagggcccagaactgctgaagctctcactgaccctctccctcacctgtgccatctctggttgctccatcaccagtgcttactggtaaccagtactccctgcagctaagctctgtgatgaccaaggacacggcagtgtgttgctgtgcaagaga

SEQ ID NO: 33 - DNA, 288 bp, Bos taurus
  source 1..288: mol_type = genomic DNA
caggtgtcctgcagcagttgggcccagaactggtgagccctcagagaccctctcctcacatgtgctatctctgcttacaccatcatgtggttatagtcagaagtggattcgccaggccgcagggaaggggctagagcagatggcatgcataaactatgatggtgacacttactacagcccctccattaagagccacacctccatctcagagacatccaagaatcagttctccctgctactgagctctgtgaccactgaggacatggccgtgtgttgctgtgcaagaga

SEQ ID NO: 34 - DNA, 288 bp, Bos taurus; identical to SEQ ID NO: 33
  source 1..288: mol_type = genomic DNA

SEQ ID NO: 35 - DNA, 296 bp, Bos taurus
  source 1..296: mol_type = genomic DNA
caggtgcagctgcaggaatcaggcccggaactgataaagtcttcacagacactctccctcacctgtgctggttctggttactccatcaccagtgattatggtaggaactggatccgccaggccccagggaagggtctagagcagatgggatgcatgtattataatggtgacacttattacagcccctccatcaagagtcacacctccatctgcagagacacacccaagaaccagttctccctgcagctgagctctgtgcccacagaggacacagccatgtgttacttggcaagaaa

SEQ ID NO: 36 - DNA, 289 bp, Bos taurus
  source 1..289: mol_type = genomic DNA
caggtgcagctggtgcagtgggggctgagctgaggaagcctggggcctcagtgaaggtgtcctgcaaggcttctggatataccttcaccgactacatgcactgggtgtgacaggcccctcagcaagagcttgaacggatggacagattgacagcaaagatggtggagcaaagtacgcacagaagttccagggcagagtcacgttggctgcagacacgtccaccagcatcacctacgtggagctgagcagtctgaggtctgacgacacggctgtttattactgtgtgaga

SEQ ID NO: 37 - DNA, 289 bp, Bos taurus; identical to SEQ ID NO: 36
  source 1..289: mol_type = genomic DNA

SEQ ID NO: 38 - DNA, 289 bp, Bos taurus; identical to SEQ ID NO: 36
  source 1..289: mol_type = genomic DNA

SEQ ID NO: 39 - DNA, 294 bp, Bos taurus
  source 1..294: mol_type = genomic DNA
caggtgcagctggtgctgttggggctgagctgaggaagcctggggcctcagtgaaggtgtcctgcaaggcttctggatacaccttcaccgactactacacgcactaggtgtgacaggcccctcagcaagggcttgaacagatggacagattgacagcaaagatggtggagcaaagtacgcacagaagttccagggcagagtcacgttggctgcagacacgtccaccagcaccgccgacatggagctgagcagtctgaggtctgaggacacggctgtttattactgtgtgagaca

SEQ ID NO: 40 - DNA, 290 bp, Bos taurus
  source 1..290: mol_type = genomic DNA
caggtgcagctggtgccgttggggctgagctgaggaagcctggggcctcagtgaaggtgtcctgcaaggcttctggatacaccttcaccgactacatgcactgcgtgtgacaggcccctcagcaagggcttgaacggatggatggactgaccctcaacatggtggaactaggtacacctagaagttccagagcagagtgatcttggttgcacacacgcccaccaacaccgcctacatggagcagagcagtctgagtctgaggacacggctgtttattactgtgtgaggta

SEQ ID NO: 41 - DNA, 291 bp, Bos taurus
  source 1..291: mol_type = genomic DNA
cagttgcagctggtgccattggggctgagctgaggaagcctggggcctcagtgaaggtgtcctgcaaggcttctggatacaccttcaccgactacatgcactgggtgtgacaggcccctcaacaagggcttgaaaggatggacagattgacagcaaagatggtggagcaaagtatgcacagaagttccagggcagagtcacgttggctgcagacacgtccaccagcaccgcctacatggagctgagcagtctgaggtctgaggacacggctgtttattactgtgtgagaca

SEQ ID NO: 42 - DNA, 291 bp, Bos taurus
  source 1..291: mol_type = genomic DNA
caggtgcagctggtgctgttgtggctgagctgaggaagcctggggcctcagtgaaggtgtcctgcaaggcttctggatacaccttcaccgactacatgcactgggtgtgacaggcccctcagcaagggcttgaagggatggacagattgacagcaaagatggtggagcaaagtatgcacagaagttccagggcagagtcacgttggctgcagacacgtccaccagcactgcctacatggagctgagcagtctgaggtctgaggacatggctgtttattactgtgtgagaca

SEQ ID NO: 43 - DNA, 289 bp, Bos taurus
  source 1..289: mol_type = genomic DNA
caggtgcagctggtgcagtgggggctgagctgaggaagcctggggcctcagtgaaggtgtcctgcaaggcttctggatacaccttcaccgactacatgcactgcgtgtgacaggcccctcagcaagggcttgaacggatggatggactgaccctcaacatggtggaactaggtacacctagaagttccagagcagagtgatcttggttgcacacacgtccaccaacaccgcctacatggagcagagcagtctgaggtctgaggacacggctgtttattactgtgtgagg

SEQ ID NO: 44 - DNA, 291 bp, Bos taurus
  source 1..291: mol_type = genomic DNA
caggtgcagctggtgccattggggctgagctgaggaagcctggggcctcagtgaaggtgtcctgcaaggcttctggatacaccttcaccgactacatgcactgcatgtgacaggcccctcagcaagggcttgaaaggatggacagattgacagcaaagatggtggagcaaagtatgcacagaagttccagggcagagtcaccttggttgcagacccgtgcacctgcactgcctacatggagctgagcagtctgaggtctgaggacacggctgtttattactgtgtgagaca

SEQ ID NO: 45 - DNA, 290 bp, Bos taurus
  source 1..290: mol_type = genomic DNA
caggtgcagctggtgcagtgggggctgagctgaggaagcctggggcctcagtgaaggtgtcctgcaaggcttctggatacaccttcaccgactacatgcactgcgtgtgacaggcccctcagcaagggcttgaacggatggatggactgaccctcaacatggtggaacaaggtacacctagaagttccagagcagagtgatcttggttgcacacacgcccaccaacaccgcctacatggagcagagcagtctgagtctgaggacacggctgtttattactgtgtgaggta

SEQ ID NO: 46 - DNA, 291 bp, Bos taurus; identical to SEQ ID NO: 44
  source 1..291: mol_type = genomic DNA

SEQ ID NO: 47 - DNA, 290 bp, Bos taurus
  source 1..290: mol_type = genomic DNA
caggtgcagctggtgccgttggggctgagctgaggaagcctggggcctcagtgaaggtgtcttgcaaggcttctggatacaccttcaccgactacatgcactgcatgtgacaggcccctcagcaagggcttgaacggatggatagattgacagcaaagatggtggagcaaagtatgcacagaagttccagggcagagtcacgttgctgcagacacgtccaccagcaccgcctacatggagctgagcagtctgaggtctgaggacacggctgtttattattgtgtgagaca

SEQ ID NO: 48 - DNA, 294 bp, Bos taurus
  source 1..294: mol_type = genomic DNA
caggtgcagctggtgcagtgggggctgagctgaggaagcctggggcctcagtgaaggtgtcctgcaaggcttctggatacaccttcaccgactactacacgcactaggtgtgacaggcccctcagcaagggcttgaacagatggacagattgacagcaaagatggtggagcaaagtacgcacagaagttccagggcagagtcacgttggctgcagacacgtccaccagcaccgccgacatggagctgagcagtctgaggtctgaggacacggctgtttattactgtgtgagaca

SEQ ID NO: 49 - DNA, 291 bp, Bos taurus
  source 1..291: mol_type = genomic DNA
caggtgcagctggtgcagtgggggctgagctgaggaagcctggggcctcagtgaaggtgtcctgcaaggcttctggatacaccttcaccgactacatgcactgcgtgtgacaggcccctcagcaagggcttgaacagatggacagattgacagcaaagatggtggagcaaagtatgcacagaagttccagggcagagtcacgttggctgcagacacgtccaccagcaccgccgacatggagctgagcagtctgaggtctgaggacacggctgtttattactgtgtgagaca

SEQ ID NO: 50 - DNA, 284 bp, Bos taurus
  source 1..284: mol_type = genomic DNA
caggtacagttggggctgagctaaggaagcctggggcctcagtgaaggtgtcctgcaaggcttctggatacaccttcaccaactactacatgcactgggtgtgacaggaccctcagcaatggcttgaatggatggacagattgacagcaaagatggtggagcaaagtatgcacagaagttccagggcagagtcacgttggctgcagacacgtccaccagcaccgcctacatggagctgagcagtctgaggtctgaggacacggctgttattactgtgtgaaaca

SEQ ID NO: 51 - DNA, 31 bp, Bos taurus
  source 1..31: mol_type = genomic DNA
agaataccgtgatgatggttactgctacacc

SEQ ID NO: 52 - DNA, 16 bp, Bos taurus
  source 1..16: mol_type = genomic DNA
ttactatagtgaccac

SEQ ID NO: 53 - DNA, 36 bp, Bos taurus
  source 1..36: mol_type = genomic DNA
gtattgtggtagctattgtggtagttattatggtac

SEQ ID NO: 54 - DNA, 43 bp, Bos taurus
  source 1..43: mol_type = genomic DNA
gtagttatagtggttatggttatggttatagttatggttatac

SEQ ID NO: 55 - DNA, 42 bp, Bos taurus
  source 1..42: mol_type = genomic DNA
atgatacgataggtgtggttgtagttattgtagtgttgctac

SEQ ID NO: 56 - DNA, 58 bp, Bos taurus
  source 1..58: mol_type = genomic DNA
gtagttgttatagtggttatggttatggttgtggttatggttatggttatgattatac

SEQ ID NO: 57 - DNA, 67 bp, Bos taurus
  source 1..67: mol_type = genomic DNA
gtagttatggtggttatggttatggtggttatggttgttatggttatggttatggttatggttatac

SEQ ID NO: 58 - DNA, 148 bp, Bos taurus
  source 1..148: mol_type = genomic DNA
gtagttgtcctgatggttatagttatggttatggttgtggttatggttatggttgtagtggttatgattgttatggttatggtggttatggtggttatggtggttatggttatagtagttatagttatagttatacttacgaatatac

SEQ ID NO: 59 - DNA, 14 bp, Bos taurus
  source 1..14: mol_type = genomic DNA
gaactcggtggggc

SEQ ID NO: 60 - DNA, 54 bp, Bos taurus
  source 1..54: mol_type = genomic DNA
actatgcagacttccatctctggagccaggctgccctgggcaccgtctcctcag

SEQ ID NO: 61 - DNA, 56 bp, Bos taurus
  source 1..56: mol_type = genomic DNA
ctgctgggacttggatctctggggccagcgcaccccggtcaccatgtccttgggga

SEQ ID NO: 62 - DNA, 50 bp, Bos taurus
  source 1..50: mol_type = genomic DNA
caatgcttttgactcctggggccagcgcacccccatctccatctcctcag

SEQ ID NO: 63 - DNA, 47 bp, Bos taurus
  source 1..47: mol_type = genomic DNA
actattcgacaactggggcccaggaatccaaaacaccgtctcctcag

SEQ ID NO: 64 - DNA, 50 bp, Bos taurus
  source 1..50: mol_type = genomic DNA
taacaactggctcaagcactggggtcaggaagcctgggcactgtctgctc

SEQ ID NO: 65 - DNA, 54 bp, Bos taurus
  source 1..54: mol_type = genomic DNA
tttactatggtatagacgcctggggccgagggctcagggtcaccgtctcctcag

SEQ ID NO: 66 - DNA, 63 bp, Bos taurus
  source 1..63: mol_type = genomic DNA
actatgctgacttccatctctgtggccaggctgccctgggcaccgtctcctcagctgaatctg

SEQ ID NO: 67 - DNA, 56 bp, Bos taurus
  source 1..56: mol_type = genomic DNA
ctgctgggacatggatctctggggccagcgcaccccggtcaccgtgtccttgggga

SEQ ID NO: 68 - DNA, 50 bp, Bos taurus
  source 1..50: mol_type = genomic DNA
caatgcttttgactcctggggccagcgcgccccggtctccatctcctcag

SEQ ID NO: 69 - DNA, 48 bp, Bos taurus
  source 1..48: mol_type = genomic DNA
actacgtcgatgcctggggccaaggactcctggtcaccgtctcctcag

SEQ ID NO: 70 - DNA, 50 bp, Bos taurus
  source 1..50: mol_type = genomic DNA
taacaactggctcaagcactggggtcgggaagcctgggcactgtctgctc

SEQ ID NO: 71 - DNA, 54 bp, Bos taurus
  source 1..54: mol_type = genomic DNA
attactatagtatatatgtttgcggccgagggatcgaggtcaccgtctcctcag

SEQ ID NO: 72 - DNA, 287 bp, Bos taurus
  source 1..287: mol_type = genomic DNA
gacatccaggtaacccagtctccatcctccttgtctgcatctctaggagacagagtctccatcacttgccaggccagtcagagcattgacactaaattagcctggtatcaacagaaaccagggaaagctcctaagctcctcatctatgcaatacccaggtcgccttcctggttcccttcccagttcagtggcagtggatttggggcagatttcaccctcaccatcagcagtctgaaggctgatgatattgcaacttactactgtcagcaggatcacggtttacctac

SEQ ID NO: 73 - DNA, 287 bp, Bos taurus
  source 1..287: mol_type = genomic DNA
gacatccaggtgacccagtctccctcctacctgtctgcttctctaggagacagagtctccatcacttgccaggccaatcagagcgttagccactacttaaactggtatcaacagaaaccaggggaagctcctaagctcctgatctattatgcaaccagccggtacaccagagtcccatcccgattcagtggcagtggatctgggacagatttcaccctcaccatcagcagcctggaggctgacgatgctgcaaattattactgtcaacaggattatagtacacctcc

SEQ ID NO: 74 - DNA, 286 bp, Bos taurus
  source 1..286: mol_type = genomic DNA
ggcatccagatgactcagtctccatcctccttgtctgcctctctaggagacagagcatccatcatttgctgggccaattaaagcattagcaaatggttagacagatatgagcagaaaccagggcaagttcctaagctcctgttctatgcagcatccaatttgggaactggggtcccatcccggttcagtggcagtagatctgggacagatttcactgtcaccactctcacctggaggctgaagatgctgcaacttattactgtctacaaactgatagtacacctcc

SEQ ID NO: 75 - DNA, 285 bp, Bos taurus
  source 1..285: mol_type = genomic DNA
gacctccagatgattcagtctctatcttccctgtctgcatctctaggagacagagtctccatcacttgtcgggccagtcaaagcgttagaaataatttacagtggtatcaagagaaaccagggaaagctcctaagttcctcatctatgacagaaccagtgtgtacacaggggtcccatcccatttcagtggcagtggatctgggacagattataccttcaccaccagcagcctgggctgatgattttgcaacttattactgtaaacaggataacagtagacctcc

SEQ ID NO: 76 - DNA, 283 bp, Bos taurus
  source 1..283: mol_type = genomic DNA
gacctccagatgacccagtctccatcctccctgtctgcatctctaggagacagaatctccatcacttgccgggccagagcgttagcaactacttagcctggtatcaacagaaaccagggaaagctcctaagctcctgatctatcacgaatccagattgcacacaggggtcccatcccggttcagtggcagtggatgtgggacagattacaccctcaccatcagcaggctggagtctgacgatgctgcaaattattactgtcagcagtataatagtacacctcc

SEQ ID NO: 77 - DNA, 302 bp, Bos taurus
  source 1..302: mol_type = genomic DNA
gatgttgtgctgacccagactccactctccctgtctatcatccctggagagatggcctccatctcctgcaagtctagtcagagcctggtacacagtgatggaaaaacctatttgaattggattcaatataaaccaggccaatcaccacagggtctgatctatcaggtttccaaccgttactctggggtctcagacaggttcactggcagtgggtcagggacagatttcacacttacaatcagcagagtgcaggctgaggatgctggagtctattactgttaccaaggtacagaagatcctcc

SEQ ID NO: 78 - DNA, 302 bp, Bos taurus
  source 1..302: mol_type = genomic DNA
gctactatgcagacccagactctacgctccctgtctgtcatcccgggagagatggcctccatctcctgcagagccagtcagagcgttcaaaatagatatggagacaattttttgcactggtatgtgcagaagcccagccagtctccacagctcctgatttatagggcttctaactgggagtcttgggtcccagacaggttcacaagcagtgggttgggaacacatttcatcctcataatcagcagggtggagtctgaggatgctggagtttattactgccagcagagtttacaagcacctcc

SEQ ID NO: 79 - DNA, 302 bp, Bos taurus
  source 1..302: mol_type = genomic DNA
gatgttgtgctgacccagactcccctctccctgtctgtcatccctggagagacggtcaccatctcctgcaagtctactcagagtctgaaatatagtgatggaaaaacgtatttgcaatggtttcaacataaaccaggccagtctccacggctattgatctatcagatttccaaccgttacactggggtcccagacaggttcactggcagtgggtcagagacagatttcacacttacaatcagcagtgtgcaggctgaggatgctggagtctattactgtcttcaaagatcatatgctcctcg

SEQ ID NO: 80 - DNA, 303 bp, Bos taurus
  source 1..303: mol_type = genomic DNA
ggctattatgcagaaccaactatacgctccctgtctgtcatccctggagagactgccttcatctcctgcagagccagtcagagcattcaatatagatagggagacaatttttttgcactggtatgtgcagaagcccagccagtctccacagctcctgatttatagggcttctaactgggagtcttgggtcccagacaggttcacaagcagtgggttgcgaacagatttcatcctcataatcagcagggtggaggctgaggatgctggagtttattactgccagcagagtttacaagcacctcc

SEQ ID NO: 81 - DNA, 302 bp, Bos taurus
  source 1..302: mol_type = genomic DNA
gatgttgtgctgacccagactcccctctccctgtctgtcatccctggagagacggtctccatctcctgcaagtctactcagagtctgaaatacagtgatggaaaaacctatttgtaccggcttcaacataaaccaggccaatcaccacagagtttgatctattatgtttccaaccgttacactggggtcccagacaggttcactggcagtgggtcagagacagatttcacacttacgatcagcagtgtgcaggctgaggatgctggagtctattactgttttcaaggcacacaggttcctcc

SEQ ID NO: 82 - DNA, 303 bp, Bos taurus
  source 1..303: mol_type = genomic DNA
gctataaggcagacccagactctacgctccctgtctgtcatccctggagagacggcctccgtctcctgcagagccagtcagagcgttcaaaatagatatggagacaatttttttgcattggtatgtgcagaagcccagccagtctccacagctcctgatctatggagcttctaaccaggcctctggagtctgagacaggttcactggcagtgggtcagggacagacttcaccctcaaaagcagcagggtcggggctgaggatgctggagtttattattgccaccaaagtaaagaaactcctcc

SEQ ID NO: 83 - DNA, 302 bp, Bos taurus
  source 1..302: mol_type = genomic DNA
gatgttgtgctgacccagactcccctctccctgtctgtcatccctggagagacggtctccatctcctgcaagtctactcagagtctgaaatatagtgatggaaaaacctatttgcgttgggttcaacataaaccaggccaatcaccacagggtgtgatctatcaggtttccaaccgtaatactggggtcccagacaggttcactggcagtgggtcagaaacagatttcacacttacaatcagcagtgtgcaggctgaggatgctggagtctattactgttttcaaggtacatatgaacctcc

SEQ ID NO: 84 - DNA, 303 bp, Bos taurus
  source 1..303: mol_type = genomic DNA
gctataatgcagacccagactctacgctccctgtctgtcatccctggagagacggcctccatctcctgcagagccagtcagagcgttcaaaatagatatggagacaatttttttgcattggtatgtgcagaagcccagccagtctccacagctcctgatctatggagcttttaaccaggcctctggagtctgagacaggttcaccggcagtgggtcagggacagatttcaccttcaaaaccagcagggtgggggctgaggatgctggagtttattattgccaccaaagtaaagaaactcctcc

SEQ ID NO: 85 - DNA, 299 bp, Bos taurus
  source 1..299: mol_type = genomic DNA
gatgttgtgctgacccagactcccctctccctgtctgtcatccctggagagacggtctccatctcctgcaagtctactcagagtctgaaatatagtggaaaaacctatttgcgttggcttcaacataaaccaggccaatcaccacagagtctgatctatcaggtttccaaccgttacactggggtcccagacaggttcactggcagtgggtcagagacagatttcacacttacgatcagcagtgtgcaggctgaggatgctggagtctattactgtgttcaagagacacatgatcctcg

SEQ ID NO: 86 - DNA, 301 bp, Bos taurus
  source 1..301: mol_type = genomic DNA
gctattgttctgacccagactccacgctccctgtctgtcatccctggagagacggcctccatctcctgcagatccagtcagagcattcaaaatagatatggagacaatcttttgcactggtatgtgcagaagcccagccagtctccacagctcctgatctatggaacttctaaccaggcctctggagtctgagacaggttcaccggcagtgggtcagggacagatttcaccctcaaaaccagcagggtggaggctgaggttgctggagtttattattgcaggaaagtaaagaaactccttc

SEQ ID NO: 87 - DNA, 302 bp, Bos taurus
  source 1..302: mol_type = genomic DNA
gatgtagtgctgacccagactccactctccttgtctgtcatccctggtgagacggcctccatctcctgcaagtcaagtcagagcctcctgcatagtgatggaaaaacctatttgaactggtttcaacataaaccaggccagtctccacagtgactgatctatcaggcttccaaccgtgacactggggtctcagagaggttcactggcagtgggtcagggacagatttcacacttaaaatcagcagagtgcagattgagtatgctggcatctattactgttttcagcatacatatgatcctcc

SEQ ID NO: 88 - DNA, 302 bp, Bos taurus
  source 1..302: mol_type = genomic DNA
gacattgtgctgacccagactccactctccttgtctgtcttccctggagagacggcgtccatctcctgcagaaccagtcagagccttgaagatagttatggagacacttatttgagttggcacttgcagaagcctagccagtctccacagcttctgatctatttggtttccaatagagcctctggggtcccagacaggttcactggcagtgggtcaggaacagatttcacctttaaaatcagcagggtggaggctgaggatgctggagtttattactgccaacagagtatacaagcacctcc

SEQ ID NO: 89 - DNA, 286 bp, Bos taurus
  source 1..286: mol_type = genomic DNA
gaaattatgttaacgcagtctccagcctccctgtctttgactccaggggaaatagccaccctcacctgcagggccagtcaaagtattagtagctacttaagactggtaccagcagaagcctgggaaggcccccagattcttcatctatgctgcctccagcagggcctctggcatcccagcccggttcggtgacagttgggtcagggacagactttactctcaccatcagcagcctggagcctgaagatgctgcagttcattcctagtgctagcataatagcgggaa

SEQ ID NO: 90 - DNA, 287 bp, Bos taurus
  source 1..287: mol_type = genomic DNA
gaggctgtgctctaccagactccagcctacatcgctgcatccctaggagagagcatctccatcacttgcagagccaatcaaagcattagtgattacttaagctggtataagcagaaacctggccaggctcctatgattctcatctatgatgctgataatcgttataatggtgtcccagagaggttcactgcgactcaatctgagacagaatttgttttcacaatcagccaagtagaggctgatgatgctgccatgtattactgccagcaggattatgcacttcctcc

SEQ ID NO: 91 - DNA, 138 bp, Bos taurus
  source 1..138: mol_type = genomic DNA
gacatcatgatgacccagtctcgaagttccttggctgagtctgcaggagaggaaggtcatcatcatctacagatccagccagaatcttctatacttcaaccagaaaacctagtttgcctggtaccagcagaaactgtg

SEQ ID NO: 92 - DNA, 285 bp, Bos taurus
  source 1..285: mol_type = genomic DNA
gctgctgtactgactccatctcctccctctggcctgtggccatggagggagcgtcgccatctcctgaaggccatctcttcccatccacagtaatggacacacctgcccgccgtgattcgggcacaaaccacacactctcctcaaccactgatcatagggattcccaggctcctgaggtcccagcctggctcagtgattgtgggtctggatggatttcacacttacactcaccagggtggcgtcccttcatgtgacttctgtgtacagaaccctcactgggaccac

SEQ ID NO: 93 - DNA, 285 bp, Bos taurus
  source 1..285: mol_type = genomic DNA
actgctgtgctgactccatctctccctctggcctgtggccatggagggagcgtcgccatctcctgaaggccatctcttctcatccacagtaatggacacaccttcccgccatgcttctggcacaaaccacacactctcctcaaccactgaccatagagggtcaccaggctcttgaggtcccagcctggctcagtgattgtgggtctggatagatttcacactcacactcaccagggtggggtccctacatgtgacttctgtgcacagaaccctcacttggaccac

SEQ ID NO: 94 - DNA, 286 bp, Bos taurus
  source 1..286: mol_type = genomic DNA
gctgctgtgctgacttcatctctccctctggcctgtggccatggagggagcatcgccatctcctgaaggccatctcttctcatccacagtaatggacacacctgcccgccatgcttctggcaaaaaccacacactctcctcaaccactgatcataggtggtccccaggcttcaggggtccaagcctggctcagtgactgtgggtctgggacggatttcacacttacacttaccagggtggggtccctacatgtgacttctgtgcacagaaccctcactgggaccac

SEQ ID NO: 95 - DNA, 284 bp, Bos taurus
  source 1..284: mol_type = genomic DNA
gctgaggagactccatctcctccctctggcctgtggccatggagggagcgccgccatctcctgaaggccatctcttctcatccacagtaatggacacacctgcccaccatgtttccggcacaaaccacacactctcctcaaccactgatcatagggcttccccaggcttcaggggtcccagcctggctcagtgactgtgggtctgggatggatttcacacttacactcaccagggtggggtctctacatgtgacttctgtgcacagaaccctcactgggaccac

SEQ ID NO: 96 - DNA, 294 bp, Bos taurus
  source 1..294: mol_type = genomic DNA
gctgctgtgctgactccgtcccctccctctggtctgcagtcgtggaaagaggcatctccatctcctgcaaggccatcccatctcatccatagaaatgaatacacctgtcctccctccttccagaacaaaccacacactctcctcacccattgacataggggtcccccaggctcctggggtcccatcctggctcagtggccatggatctgggacggatttcacactcacactcaccactgtggagactggggaccctgaatgtgacttctgtgcacagagccttcaatgggaact

SEQ ID NO: 97 - DNA, 38 bp, Bos taurus
  source 1..38: mol_type = genomic DNA
atggacgttaggtcaaggaaccaagctggaagtcaaac

SEQ ID NO: 98 - DNA, 39 bp, Bos taurus
  source 1..39: mol_type = genomic DNA
taaatactttcggccaaggaaccaaggtagagatcaaaa

SEQ ID NO: 99 - DNA, 38 bp, Bos taurus
  source 1..38: mol_type = genomic DNA
gttcactttcgggccaaggaccagagtggagatcaaat

SEQ ID NO: 100 - DNA, 38 bp, Bos taurus
  source 1..38: mol_type = genomic DNA
aattacgttcggcggcgggaccaaggtggaaatcaatc

SEQ ID NO: 101 - DNA, 38 bp, Bos taurus
  source 1..38: mol_type = genomic DNA
gatcatctttggccaagggacacgtctggagattagac

SEQ ID NO: 102 - DNA, 296 bp, Bos taurus
  source 1..296: mol_type = genomic DNA
caggctgtgctgactcagccgccctccgtgtccgggtccctgggccagacggtcaccatctcctgcaccggaagcagcaacaacatcgggattttgggtgtgagctggtaccaacagatcccaggatcggcccccagaaccctgatctataatagtaacaaacgaccctcgggggtccccgaccgattctctggcaccaagtccggcaacacaggcaccctgaccatcgcttcgctccaggctgaggacgaggctgattattactgtgcgtctgctgacctcagtcttactagtcc

SEQ ID NO: 103 - DNA, 291 bp, Bos taurus
  source 1..291: mol_type = genomic DNA
caggctgtgctgactcagcagccctccgtttccgggtccctgggccagagggtctccatctcctgctctggaagcagcagcaacattgggcatggttatggtacctggtaccaacagatcccaggatcggcccccagaatgctcatctatggtgcgaccagtcgagcctccggtccccgaccgattctccggctccaggtctggcaacacagcgactctgaccatcagctcgctccaggctgaggatgaggcggattatttctgtgcagcttatgacagtagcagtggtcc

SEQ ID NO: 104 - DNA, 299 bp, Bos taurus
  source 1..299: mol_type = genomic DNA
caggatgtgctgactcagccgtcctccgtgtccgggtccctgggtcagaaggtctccatcacctgctctggaagcagcagcaacgttggatatgccaattatgtgagctggcaccaacagaaaccaggatcggcccccagaaccctcatctatggtgcgaccagtcgagcctcgggggtccctgaccaattctccggctccaagtctggcaacacagcgactctgaccatcagctcgctccagcctgaggacgaggctgattattactgttcatcttatgacagtagcagcaatattgg

SEQ ID NO: 105 - DNA, 291 bp, Bos taurus
  source 1..291: mol_type = genomic DNA
caggctgtgctgactcagccgccctccgtgtctgggactttgggtcagagggtcaccctctcctgcactggaagcagcagcaacactggggtctttatgtgagctggtaccaacagctcccaggaaggcccccagagtcctgacctatgaaaatagcaaacgaacctcaggactcccagattgattctctggctccaagtctggcagctcggccgcactgaccacctcagttcagtctgaggacgacactgattattactgtttctcatgggctgatggattgaaagtttg

SEQ ID NO: 106 - DNA, 292 bp, Bos taurus
  source 1..292: mol_type = genomic DNA
caggctgtgctgactcagccgccctccgtgtccaggactttgggtcagagggtcaccctctcctgcactggaagcagcaacaaccctggggttattctgtgagctggtaccaacagctcccaggaaaggcccccacacttctcatctatgaaaatagcacacgaccctcagcactcccagattgattctctggctccaagtctggcaagtcggtctctctgaccacctcagttcagtctgaggacgacactgattattactgtttctcatgggctgacggattgaaagtttg

SEQ ID NO: 107 - DNA, 296 bp, Bos taurus
  source 1..296: mol_type = genomic DNA
caggctgtgctgactcagccgtcctccgtgtccggctccctgggccagagggtctccatcacctgctctggaagcagcaacaacatcggtagttatggtgtgggctggtaccaacaggtcccaggatcgggcctcagaaccatcatctatggtagtagcagtcgaccctcgggggtccccgaccgattctccggctccaagtctggcaacacagccaccctgaccatcagctcgctccaggctgaggacgaggcggattatttctgtgcaactgttgactacagtagcagtactgt

SEQ ID NO: 108 - DNA, 287 bp, Bos taurus
  source 1..287: mol_type = genomic DNA
caggctatgctgactcagctgccctccatgtccgggactttgggtcagagggtcaccctctcctgcactgaaagcagcagcaaccctggggtctttatgtgagctggtaccaacagctcccaggaaaggcccccagagtcctgacctgtgaaaatagcaaacgaccctcaggggtcccagattgattctctggctccaagtctggcaacagcctctcttaccacctcagttcatgctgaggatactgattactactgtttctcatgggctgacggcttgaaagtttg

SEQ ID NO: 109 - DNA, 295 bp, Bos taurus
  source 1..295: mol_type = genomic DNA
caggctgtgctgactcagccgtcctccgtgtccgggtccctgggccagagggtctccatcacgtgctctggaagcagcagcaacgttggatatggcaattatgtgagctggttccaagacatcccaggatcggcccccagaaccctcatctatggtgacaccagtcgagcctcgggggtccccgaccgattctccggctccaggtctgggaacacagccaccctgaccatcagctcgctccaggctgaggacgaggcagattatttctgtgcatcttatcagagtggtaacacag

SEQ ID NO: 110 - DNA, 295 bp, Bos taurus
  source 1..295: mol_type = genomic DNA
caggctgtgctgactcagccatcatccgtgtccgggtccctgggccagagggtctccatcacctgctctggaagcagcagcaatgttggaaatggatatgtgagctggtaccaactgatcccaggatcggcccccagaaccctcatctatggtgacaccagtcgagcctcgggggtccccgaccgattctccggctccaggtctggaacacagccaccctgaccatcagctcgctccaggctgaggacgaggcagattatttctgtgcatctgctgaggatagtagcagtaatgc

SEQ ID NO: 111 - DNA, 291 bp, Bos taurus
  source 1..291: mol_type = genomic DNA
caggctatgctgactcagccgccctccatgttcgggactttgggtcagagggttaccctctccttcactggaaggagcagcaacactgggggtctttatgtgagctggtaccaacagctcccaggaaaggcccctagactcctgacatatgaaaatagcaaacgaccctcaggggtcccagattgattctctggctccaagcctgccaactcagcctctctgaccacctcagttcatgctgaacgatactgattattactgtttctcatgggctgatggcttgaaagtttg

SEQ ID NO: 112 - DNA, 295 bp, Bos taurus
  source 1..295: mol_type = genomic DNA
caggctgtgctgactcagccgtcctccgtgtccgggtccctgggccagagggtctccatcacctgctctggaagcagcagcaacgttggaactggcaattatgtgagctggttccaacagatcccaggatcggcccccagaaccctcatctatggtgcgaccagtcgagcctcgggggtccccgaccgattctccggctccaggtctgggaacacagccaccctgaccatcagctcgctccaggctgaggacgaggcagattatttctgtgcatcttatcagagtggtaacacag

SEQ ID NO: 113 - DNA, 299 bp, Bos taurus
  source 1..299: mol_type = genomic DNA
caggctgtgctgactcagccgtcctccatgtccgggtccctgggccagagggtctccatcaccagctctggaagcagcagcaacgttggatatggcatttatgtgaaccagtaccaaaaaatcccaggatcggcccccagaaccctcatctatggtgccaccagtcgagcctcgggggtccccgaccgattctccggctccaggtctgggaacacagccaccctgaccatcagctcgctccaggctgagaacgaggcagattatttctgtgcagcttatgacagcagtagcagtgatgg

SEQ ID NO: 114 - DNA, 299 bp, Bos taurus
  source 1..299: mol_type = genomic DNA
caggctgtgctgactcagccgtcctccgtgtccgggtccctgggccagagggtctccatcacctgctctggaagcagcagcaacgttgggcttggtaattatgtgagctggttccaacagatcccaggatcggcccccagaaccctcatctatggtgcgaccagtcgagcctcgggggtccccgaccgattctccggctccaggtctgggaacacagccaccctgaccatcagctcgctccaggccgaggacgaggcggattatttctgtgcatctcctgacagtagtagcagtagtta

SEQ ID NO: 115 - DNA, 291 bp, Bos taurus
  source 1..291: mol_type = genomic DNA
caggctatgctgactcagccgccctccatgttcgggactttgggtcagagggttaccctctccttcactggaaggagcagcaacactgggggtctttatgtcagctggtaccaacagctcccaggaaaggcccctagactcctgacatatgaaaatagcaaacgaccctcaggggtcccagattgattctctggctccaagcctggcaactcagcctctctgaccacctcagttcatgctgaacgatactgattattactgtttctcatgggctgatggcttgaaagtttg

SEQ ID NO: 116 - DNA, 295 bp, Bos taurus
  source 1..295: mol_type = genomic DNA
caggctgtgctgactcagccgtcctccgtgtccgggtccctgggccagagggtctccatcacgtgctctggaagcagcagcaacgttggatatggcaattatgtgagctggttccaagagatcccaggatcggcccccagaaccctcatctatggtgacaccagtcgagcctcgggggtccccgaccgattctccggctccaggtctgggaacacagccaccctgaccatcagctcgctccaggctgaggacgaggcagattatttctgtgcatcttatcagagtggtaacacag

SEQ ID NO: 117 - DNA, 299 bp, Bos taurus
  source 1..299: mol_type = genomic DNA
caagctgtgctgactcaaccgccctccatgtctgggtccctgggccagagggtctccatcacctgctctggaagcagcagcaacgttggaactggcaattatgttggctggtaccaaatgatcccaggatcggcccccagaaccctcatctaccgtgctaccagtcgactctcgggggtccccgactgattctccgtctccaggtctgggaacacagccaccctgaccatcagctcgcaccaggctgaggacgaggctgattattactgtgtatcttaggacagcagtatcagtggtgc

SEQ ID NO: 118 - DNA, 296 bp, Bos taurus
  source 1..296: mol_type = genomic DNA
caggctgtgctgactcagccatcatccgtgtccgggtccctgggccagagggtctccatcacctgctctggaagcagcagcaatgttggaaatggatatgtgagctggtaccaactgatcccaggatcggcccccagaaccctcatctatggtgacaccagtcgagcctcgggggtccccgaccgattctccggctccaggtctgggaacacagccaccctgaccatcagctcgctccaggctgaggacgaggcagattatttctgtgcatctgctgaggatagtagcagtaatgc

SEQ ID NO: 119 - DNA, 291 bp, Bos taurus; identical to SEQ ID NO: 111
  source 1..291: mol_type = genomic DNA

SEQ ID NO: 120 - DNA, 299 bp, Bos taurus
  source 1..299: mol_type = genomic DNA
caagctgtgctgactcaaccgccctccatgtctgggtccctgggccagagggtctccatcacctgctctggaagcagcagcaacgttggaactggcaattatgttggctggtaccaaatgatcccaggatcggcccccagaaccctcattgaccgtgctaccagtcgactctcaggggtccccgactgattctccgtctccaggtctgggaacacagccaccctgaccatcagctcgcaccaggctgaggacgaggctgattattactgtgtatcttacgacagcagtatcagtggtgc

SEQ ID NO: 121 - DNA, 296 bp, Bos taurus; identical to SEQ ID NO: 118
  source 1..296: mol_type = genomic DNA

SEQ ID NO: 122 - DNA, 291 bp, Bos taurus; identical to SEQ ID NO: 111
  source 1..291: mol_type = genomic DNA

SEQ ID NO: 123 - DNA, 295 bp, Bos taurus
  source 1..295: mol_type = genomic DNA
caggctgtgctgactcagccgtcctccgtgtccgggtccctgggccagagggtctccatcacctgctctggaagcagcagcaacgttggaactggcaattatgttggctggttccaacagatcccaggatcagcccccagaaccctcatctatggtgcgaccagtcgagcctcgggggtccccgaccgattctccggctccaggtctgggaacacagccaccctgaccatcagctcgctccaggctgaggacgaggcagattatttctgtgcatcttatcagagtggtaacacag

SEQ ID NO: 124 - DNA, 291 bp, Bos taurus
  source 1..291: mol_type = genomic DNA
caggctgtgctgactcagccgccctccgtgtctgggactttgggtcagagggtcaccctctcctgcactggaagcagcagcaaccctggggtctttatgtgagctggtaccaacagctcccaggaaggcccccagagtcctgacctatgaaaatagcaaacgaccctcaggactcccagattgattctctggctccaagtctggcagctcggccgcgctgaccacctcagttcagtctgaggacgacactgattattactgtttctcatgggctgatggcttgaaagtttg

SEQ ID NO: 125 - DNA, 296 bp, Bos taurus
  source 1..296: mol_type = genomic DNA
caggctgtgctgactcagccatcatccgtgtccgggtccctgggccagagggtctccatcacctgcaccggaagcagcagcaatgttggaaatggatatgtgagctggttccaacagatcccaggatcggcccccagaaccctcatctatggtgacaccagtcgagcctcgggggtccccgaccgattctccggctccaggtctgggaacacagccaccctgaccatcagctcgctccaggctgaggacgaggcagattatttctgtgcagctggtgacagcagtagcagtaatgc

SEQ ID NO: 126 - DNA, 291 bp, Bos taurus
  source 1..291: mol_type = genomic DNA
caggctatgctgactcagccgccctccgtgtttgggactttgggtcagagggttaccctctccttcactggaaggagcagcaacactgggggtctttatgtgagctggtaccaacagctcccaggaaaggcccctagactcctgacatatgaaaatagcaaacgaccctcaggggtcccagattgattctctggctccaagcctggcaactcagcctctctgaccacctcagttcatgctgaatgatactgattattactgtttctcatgggctgatggcttgaaagtttg

SEQ ID NO: 127 - DNA, 298 bp, Bos taurus
  source 1..298: mol_type = genomic DNA
caggctgtgctgactcagccatcatccgtgtccgggtccctgggccagagggtctccatcacctgctctggaagcagcagcaatgttggaaatggatatgtgagctggtaccaactgatcccaggatcggcccccagaacccttcatctatggtgacaccagtcgagcctcgggggtccccgaccgattctccggctccaggtctgggaacacagccacccctgaccatcagctcgctccaggctgaggacgaggcagattatttctgtgcatctgctgaggatagtagcagtaatgc

SEQ ID NO: 128 - DNA, 298 bp, Bos taurus
  source 1..298: mol_type = genomic DNA
caagctgtgctgactcaaccgccctccatgtctgggtccctgggccagagggtctccatcacctgctctggaagcagcagcaacgttggaactggcaattatgttggctggtaccaaatgatcccaggatcggcccccagaaccctcatctaccgtgctaccagtcgactctcggggtccccgactgattctccgtctccaggtctgggaacacagccaccctgaccatcagctcgcaccaggctgaggacgaggctgattattactgtgtatcttaggacagcagtatcagtggtgc

SEQ ID NO: 129 - DNA, 293 bp, Bos taurus
  source 1..293: mol_type = genomic DNA
caggctgggctaactcagccggcctccgtgttcaggactttgggtcagagggtcaccatctcttgtactggaagcagcaacaacattgggggttattatgtgagctggtaccaacagctcccaggaaaggcccccagactcctgacctatgaaattagcaaacgacccccaggggtcccagatcgagtctctggctccaagtctggcaactcagcctctctgaccagctcagttcatgctgaggacgacactgattattactgtttctcatgggctgacggcttgaaagtttg

SEQ ID NO: 130 - DNA, 299 bp, Bos taurus
  source 1..299: mol_type = genomic DNA
caggctgtgctgacccagccgccctccgtgtccgggtccctgggccagagggtgaccatctcctgcactggaagcagcagcaacatcggtggtggtaattgtgtgggctggtaccaacagatcccaggatcggcccccaaaaccctcatctataggagtaccagtcgaccctcgggggtcccagaccgattctccggctccaggtctggcaacacggccaccttgaccatcagctcgctccaggccgaagacgaggcggattactactgtgcaacttacgaaagtagtagttatcatgg

SEQ ID NO: 131 - DNA, 291 bp, Bos taurus
  source 1..291: mol_type = genomic DNA
caggctatgctgactcagccgccctccgtgttcgggactttgggtcagagggttaccctctccttcactggaaggagcagcaacactgggggtctttatgtcagctggtaccaacagctcccaggaaaggcccctagactcctgacatatgaaaatagcaaacaaccctcaggactcccagattgactctctggctccaagcctggcaactcagcctctctgaccacctcagttcatgctgaacgatactgattattactgtttctcatgggctgacggcttgaaagtttg

SEQ ID NO: 132 - DNA, 236 bp, Bos taurus
  source 1..236: mol_type = genomic DNA
acctgctctggaagcagcaacaacatcggtagatatggtgtgggctggtaccaacaggtcccaggatcgggcctcagaaccatcatctatggtagtagcagtcgaccctcgggggtccccgaccgattctccggctccaagtctggcaacacagccaccctgaccatcagctcgctccaggctgaggacgaggcggattatttctgtgcaactggtgactacagtagcagtactgt

SEQ ID NO: 133 - DNA, 299 bp, Bos taurus
  source 1..299: mol_type = genomic DNA
caggctgtgctgacccagccgccctccgtgtccgggtccctgggacagagggtgaccatctcctgcactggaagcagcagcaacatcggtggtggtaattatgtgggctggtaccaacagatcccaggatcggcccccaaaaccctcatctataggagtaccagtcgaccctcgggggtcccagaccgattctccggctccaggtctggcaacacggccaccttgaccatcagctcgctccaggccgaagacgaggcggattactactgtgcaacttacgaaagtagtagttatcatgg

SEQ ID NO: 134 - DNA, 293 bp, Bos taurus
  source 1..293: mol_type = genomic DNA
caggctgtgctgactcagctgccctccgtgttcaggactttgggtcagagggtcaccatctcttgtactggaagcagcaacaacattgggggttattatgtgagctggtaccaacagctcccaggaaaggcccccagactcctgacctatgaaattagcaaacgacccccaggggtcccagatcgagtctctggctccaagtctggcaactcagcctctctgaccagctcagttcatgctgaggacgacactgattattactgtttctcatgggctgacggcttgaaagtttg

SEQ ID NO: 135 - DNA, 299 bp, Bos taurus
  source 1..299: mol_type = genomic DNA
caggctgtgctgactcagccgccctccgtgtccgggtccctgggccagagggtgaccatcacctgcaccggaagcagcagctacgtttcgcgtggcaatcatgtgagctggtaccaactgatcccaggattggcccccaaaaccctgatctataatagtaacaaacgaccctcgggggtccctgaccgattctctggcaccaagtccggcaacacaggcaccctgaccatcgcttcgctccaggctgaggacgaggctgattattactgtgcgtctgctgacctcagtcttactggtcc

SEQ ID NO: 136 - DNA, 297 bp, Bos taurus
  source 1..297: mol_type = genomic DNA
cagtctggcctgactcagccttcctcagtgtctgggaatctgggacagacggtcaccatctcctgtgctgggaccagcagtgatgtaggggcttataatggtgtgggctggtaccaacagctcccgggctcagcccccaaaactctgatctataatctcaacaaacggtcctcagggatccctgctcggttctctggctccaagtctgggaacacagccaccctgaccatctctgggctccaggctgaggacgaggccgactattactgtagctcatataaaagtggtggtagtgtg

SEQ ID NO: 137 - DNA, 297 bp, Bos taurus
  source 1..297: mol_type = genomic DNA
cagtctagcctgactcagccttcctcagtgtctgggaatctgggacagacggtcaccatctcctgtgctgggaccagctgtgacgtagggagttataatggtgcgggctggtaccaacagctcccgggctcagcccccaaaactctgatatgtaatgtcagcaaacggccctcagggatccctgactggttctctggctccaagtccggaaacacagccaccctgaccatctctgggctccaggctgaggacgaggctgattactattggagctctcctagaagtgatagcactgtg

SEQ ID NO: 138 - DNA, 295 bp, Bos taurus
  source 1..295: mol_type = genomic DNA
cagtctggcctgactcagcctccctcagtgtctgggaatctgggacagacggtcaccagctcctgttctgagaccagcagtgacatcatggttataactctgtagattggtactggcagcacttgggcacggccccacactactgatttatgctgtcagtaaacgaccctcagggatccctgatcgcttctctggctccaagcctggacacacagcctccctgactgtctctgggctccaggctgaggacgaggctgattatcactgtggctcagacagaagcagcaaccacttg

SEQ ID NO: 139 - DNA, 297 bp, Bos taurus
  source 1..297: mol_type = genomic DNA
cagtctggcctgactcagccttcctcagtgtctgggaatctgggacagactgtcatcacctcctgtgctgggaccagcagttatgtagggagttataatggtgtgggctggtaccaacagctcccgggctcagcccccaaaactctaatatataatgtcagcaaacggccctcaggaatccctgaccgcttctctggctccaagtccgggaacacagccaccctgaccgtctctgggctccaggctgaggacgaggccgactactactgtagctcatataaaagtggtggtagtgtg

SEQ ID NO: 140 - DNA, 291 bp, Bos taurus
  source 1..291: mol_type = genomic DNA
tcctacgagctgactcagtcacccccggcatcgatgtccccaggacagacggccaggatcacgtgtggggggcccagcgttggaggtgaaaatgttgagtggcaccagcagaagccaggccaggcccgtgcgctggtcacctatggtgacgataaccgacccacgggggtccctgaccagttctctggcgccaactcagggaacatggccaccctgaccatcagcggggcccgggccaaggatgaggccgactattactgtcagctgtgggacagcagcagtaacaatcct

SEQ ID NO: 141 - DNA, 285 bp, Bos taurus
  source 1..285: mol_type = genomic DNA
tcttctcagctgactcagccgcctgcggtgtccgtgtccttgggacagacagccagcatcacctgccagggagacgacttagaattgcttagtgcccactggtaccagcagaagccgggccaggcccctgtgctggtcatttatgcagatgacaacctggcctcagggatccctgaccggttctctggctccaaatcagacaccacggccaccctgaccattcgcggggcccaggccgaagacgaggccgactattattgtcagtcagctgatatcagtggtgtt

SEQ ID NO: 142 - DNA, 291 bp, Bos taurus
  source 1..291: mol_type = genomic DNA
tcctatgaactgacacagttgacttcagtgtcagtggccttgggacagacggccaagatcacctgctcgggggagctgctggatgaacaatatactcagtggtaccagcagaagccgggccaggcccctaagctggtcatttataaagacagtaagcggcgctcagggatccctgaccagttctctggctccagctccggcaaaacagccatcttgaccatcagtggggtccgtgccgaggatgaagccgactattactgtctgtcgtgggacagtggcagttacaatgtt

SEQ ID NO: 143 - DNA, 288 bp, Bos taurus
  source 1..288: mol_type = genomic DNA
tcctatgaactgacccagccgacttcagtgtcagtggccttgggacagacggccaagatcacctgctcgggggacctgctggatgaacaatatactcagtggtaccagcagaagccgggccagggccctgtgagggtcatttataaagatagtgagcggccctcagggatctctgaccggttctctggctccagctcaggcaaaacagccacgctgaccatcagcggggcccagaccgaggacgaggccgactattactgtcagtcagctgacagcagtgataatcct

SEQ ID NO: 144 - DNA, 288 bp, Bos taurus
  source 1..288: mol_type = genomic DNA
tcttctcagctgactcagccgcctgcggtgtccgtgtccttgggacagacggccagcatcacctgccagggagacgacttagaaagctattatgctcactggtaccagcagaagccaagccaggcccctgtgctggtcatttatgagtctagtgagagaccctcagggatccctgaccggttctctggctccagctcagggaacacggccaccctgaccatcagcggggcccagactgaggacgaggccgactattactgtcagtcatatgacagcagcggtgatcct

SEQ ID NO: 145 - DNA, 308 bp, Bos taurus
  source 1..308: mol_type = genomic DNA
cagcctgtgctgactcagccagccaccctctctgcgtctctgggagcatcagccaaactcaccggcaccctgagcagtggctacaatgttggcagctactacataaactggtaccagcagaagccagggagtcctccctggtacccctgtattgttactcagactccaataagcaccagggttccagggtccccagccacttctttggatccaaagacacctcggtgaaggcagggctcctgctaatctcggctacaggctgaggacaaggctgactattactctgctacatattgcagtagtactaa

SEQ ID NO: 146 - DNA, 315 bp, Bos taurus
  source 1..315: mol_type = genomic DNA
cagcgtgtgctgactcagccggcctccccctctgcgtctccgggagcatcagccagactcccagactgcaccctgaacagtgggtctatcttggtggctagcaaatgtcctgtttccagcagaagccagggagccctccccaggacctcctgatgttcaagtcagactccgataagccccagggctccggggtccccagtcacttctctggatccaaggctgcctcagccaatgcagggcccccgttcatctctgggctgcagcctgaggctgaggctgattataactgctactgtccccaaaacactgcattca

SEQ ID NO: 147 - DNA, 285 bp, Bos taurus
  source 1..285: mol_type = genomic DNA
cagcctgtgctgactcagtcagactccctgtctgcatctctgggagcatcagccagactctcctgcaccctgagcaatggctataacattggcagcttgtctataacctggtgccagcagaagccagggagtcctccccggtacctcctgtcctacaactcagattcccaaaagctccagggctccggggtccccagacacttctctggatccaaagacacctcgtccaacgcggggctcctgctcatctctgggctgcagacgggggacgaggctgtaggttcc

SEQ ID NO: 148 - DNA, 285 bp, Bos taurus
  source 1..285: mol_type = genomic DNA
cagcctgtgctgactcagtcagactccctgtctgcatctctgggagcatcagccagactctcctgcaccctgagcaatggctataacattggcagcttgtctataacctggtgccagcagaagccagggagtcctccccggtacctcctgtcctacaactcagattcccaaaagctccagggctccggggtccccagacacttctctggacccaaagacacctcgtccaacgcggggctcctgctcatctctgggctgcagacggaggacgaggctgtaggttcc

SEQ ID NO: 149 - DNA, 317 bp, Bos taurus
  source 1..317: mol_type = genomic DNA
cagcctgtgctgactcagccgtcgccgtctctgcgtctctgggagcatcagccagactctcctgcaccctgagcagtggctacaatgttagcaactatagcaatatactggtatcagcagaaggcagggaaccctctccggtacctcctgaggttcaaatcagactcggataaacaccagggctccggggtccccagccgcttctctggatccaaagatgcctcgaccaatgcagggctcctgctcatctctgggctgcagcccgaggacgaggccgactactactgtgctgtgtggcatggcgacactaacgctta

SEQ ID NO: 150 - DNA, 317 bp, Bos taurus
  source 1..317: mol_type = genomic DNA
cagcctgtgctgactcagccagtcaccgtctctgcgtctctgggagcatcagccagactctcctgcaccctgagcagtggctacaatgttagcaactatagcatatactggtatcagcagaaggcagggaaccctctccggtacctcctgaggttcaaatcagactcggataaacaccagggctccggggtccccagccgcttctctggatccaaagatgcctcgaccaatgcagggctcctgctcatctctgggctgcagcccgaggacgaggccgactactactgtgctgtgtggcatggcgacactaacgctta

SEQ ID NO: 151 - DNA, 314 bp, Bos taurus
  source 1..314: mol_type = genomic DNA
cagcctgtgctgactgagccggcatccccctctgcatatccaggagcatcagccagactcacctgcaccctgagcagtgggtaccgtgttggtggctaccaaatgtcctgtttccagcagaaggcagggagccctccctggtacctcctgatgttcaagtcagactcggataagccccagggctctggggtccccagtcacttctctggatccaaggctgcctcagccaacacagggctcctgctcatctccgggctgcagactcaggatgaggctgattataactgctactgtccccgaaacactggtattta

SEQ ID NO: 152 - DNA, 292 bp, Bos taurus
  source 1..292: mol_type = genomic DNA
cagactgtggtccaggagccagcgctgtcagtgtgtccagtagggacggtcaccctcaccggtggactgagctctgggtcagtcactaccagtaactgcccagctggtaccagcagaccccgggccaggctccccgactgcttatctacagcacaagcagccgatattctggggtccctgctcacttctctggctccatctctggaaacaaatccaccctcaccatctcgggggcccagtccgaggtagaagccgactattactgtggtctgggaactggtagttacaatgc

SEQ ID NO: 153 - DNA, 292 bp, Bos taurus; identical to SEQ ID NO: 152
  source 1..292: mol_type = genomic DNA

SEQ ID NO: 154 - DNA, 293 bp, Bos taurus
  source 1..293: mol_type = genomic DNA
tagactgtggcccagaagccgtcacggccagtgtctccaggagagacggtcaccctcacctgtggactgagctctgggtcagtcacaaccagtaactaccctagctggttgcagcagaccccaggccaggctccctgactgcttttctatagcacaaacagtcgcccgtctggggtctctaattgcatctctggttccatctctgggaacaaagccaccctcaccatcacgggggcccagtccgaggacgaagccgattatcactgtggtctgggaactggtagttacaatgc

SEQ ID NO: 155 - DNA, 292 bp, Bos taurus
  source 1..292: mol_type = genomic DNA
cagactgtggtccaggagccagcactgtcagtgtgtccaggagggacggtcaccctcacctgtggactgagctctgggtcagtcactaccagtaactgcccagctggtaccagcagaccccaggccaggctccccgactgcttatctacagcgcaagcagctgatattctggggtccctgcttacttctctggctccatctcgggaaacaaatccaccctcaccatctcgggggcccagtccgaggtagaagccgactattactgtggtctgggaactggtagttacaatgc

SEQ ID NO: 156 - DNA, 292 bp, Bos taurus
  source 1..292: mol_type = genomic DNA
gcagcagtggcccagaagccgtcacggtcagtgtgtccaggaggcacggtcaccctcacctgtggactgagctctgggtcggtcactacaggtaaccacccagctggttccagcagaccccagtgcagcctcccggaactgtcaactacaacaccaacacccgtccctctggggtccctggtaacttctctggctcctcctctgggagcagatctgccctcaccatcacaggagaccagtccgaggacaaagccaactatcactgtgctctgggagctagtagttaaaatcc

SEQ ID NO: 157 - DNA, 299 bp, Bos taurus
  source 1..299: mol_type = genomic DNA
cagattgtgatccaggaaccgtcactgtcagtgtctccaggagggacggtcaccctcacctgtggactgagctctgggtcagtcactacttacaacgaacccagctggtaccagcagaccccaggccaggctcccagaaatgttatctacaacacaaacacccgcacctctggggtccctgatcgcttctctgcctccatctctgggaacaaagccaccctcaccatcacgggggcccagcccaaggacgaggctgactatcactgcttgctgtaccagggcagtggtagttacagctg

SEQ ID NO: 158 - DNA, 293 bp, Bos taurus; identical to SEQ ID NO: 154
  source 1..293: mol_type = genomic DNA

SEQ ID NO: 159 - DNA, 293 bp, Bos taurus
  source 1..293: mol_type = genomic DNA
tagactgtggcccagaagccgtcacggccagtgtctccaggagagaaggtcaccctcacctgtggactgagctctgggtcagtcacaaccagtaactaccccagctggttgcagcagaccccaggccaggctccctgactgcttttctatagcacaaacagtcgcccgtctggggtctctaattgcatctctggttccatctctgggaacaaagccaccctcaccatcacgagggcccagcccaaggacgaagccgattatcactgtggtctgggaagtggtagttacaatgc

SEQ ID NO: 160 - DNA, 294 bp, Bos taurus
  source 1..294: mol_type = genomic DNA
tagaactgtggcccagaagccgtcacggccagtgtctccaggagagaaggtcaccctcacctgtggactgacctctgggtcactcacaaccagtaactaccccagctggttccagcagaccccaggccaggctccctgattgctttcctatagcacaaacagtcgtccgtctggggtttctaattgcatctctggttccatctctgggaacaaaaccaccctcaccatcaaggtggcccagcccaaggacgaagccgattatcactgtggtctgggaactggtagttacaatgc

SEQ ID NO: 161 - DNA, 293 bp, Bos taurus
  source 1..293: mol_type = genomic DNA
caatccgggctgactcaggaggcctccgtgtcacggtctctgggtcagtcggtcaccctcacctgcactgggagcagcaacaacgttggattctatggcgcgggctggtcccaacaccgcccaggtgctgcccccagaaccgtggtgctgggaagttctcgaccctcaggcctcccagcccggctctcgggctcctgttctggctccaccacctcactgagcatctctgggctccaggctgcggacgaggctgactattactgttccctgtgggcccgcagcctcagtgctcc

SEQ ID NO: 162 - DNA, 176 bp, Bos taurus
  source 1..176: mol_type = genomic DNA
gtgtctttgtatcaggagaacccaggctctgccctaaaatctctgatttatgatgtcagtaaaaggtcctcaggggtcctgtttgcttctcaggctcaaactctgggaacaccctggccacctctgggctccaggctgactcttattgtggctcacatgaaagtggacgcaatttg

SEQ ID NO: 163 - DNA, 244 bp, Bos taurus
  source 1..244: mol_type = genomic DNA
tatggacgctcagccacactcgcctgcctgggaacagcaacactgttggcaccaagggggcgacttggctgccgtctcagtcgtgctgagtcccaagctctgagcacaggagtcacaacccacccgcagggtctcagcgaggcctgagggctccgggtcaggtggggccacctgaccatctctgggctccagcctgacgccaaggctgattgttcctgctcagctgggactcagccctgctgtt

SEQ ID NO: 164 - DNA, 245 bp, Bos taurus
  source 1..245: mol_type = genomic DNA
tgcaccctgagcagtgacatcagtgtcggctgctctgctgttactggaacaagcagcagccagggagccctcttcggtcctctggtcctaccactcagactccagtaagaaccaggctctggggtccccgtgggttttctggatccaaagatgccttggccaacgtggggctcctgctcgtctctgggctgcagcctgaggatgaggctgactctcaccatgcaggctggtgcaacagggcttct

SEQ ID NO: 165 - DNA, 245 bp, Bos taurus
  source 1..245: mol_type = genomic DNA
tgtaccctgagcagtgacatcagtgtcggccactctgctgttactggagccggcagaagccagcgagccctcctcggtcctccggtcctaccgctcagactccagtaaggaccaggctccagggtccccgtgggttttctggatccaaagatacctcggccaacgtgggcctcctgctcatctctgggctgcagcctgagcatgaagctgactctgaccatgcaggctggtgcaacagggcttct

SEQ ID NO: 166 - DNA, 245 bp, Bos taurus
  source 1..245: mol_type = genomic DNA
tgcaccccgagcagtgacatcagtgttggctgctctgctgttactggaaccagcagaagccagcgagccctccttagtcctccagtcctaccactcagactccagtaagaaccagtctttggggtccccgcgggttttctggatccaaagatgcctcagccaacgcggggctcctgctcgtctctgggctgcagcctgaggatgaggctatctctaaccatgcaggctggtgcaacagggcttct

SEQ ID NO: 167 - DNA, 245 bp, Bos taurus
  source 1..245: mol_type = genomic DNA
tgcaccctgagcagtgacatcaatgttggctgctctgctgttactggaaccagcagaagccagcgagccctccttagtcctccggtcctaccactcagactccagtaagaaccagtctttggggtccccgcgggttttctggatccaaagatgcctcagccaacgcggggctcctgctcgtctctgggctgcagcctgaggatgaggctatctctaaccatgcaggctggtgcaacagggcttct

SEQ ID NO: 168 - DNA, 245 bp, Bos taurus
  source 1..245: mol_type = genomic DNA
tgcaccctgagcagtgacatcagtgtcggccgctctgctgttactggaaccagcagaagccagcgagccctcctcggtcctccggtcctaccactcagattccagtaagaaccaggctccggggtccccatgggttttctggatccaaagatgcctcggccaatgcggggctcctgctcgtctctgggctacagcttgaggatgaggctgactctgaccatgcaggctggtgcaacagggctcct

SEQ ID NO: 169 - DNA, 246 bp, Bos taurus
  source 1..246: mol_type = genomic DNA
tgcacccggagcagtgacatcagtgtcggccgctctgctgttactagaaccagcagaagccagtgagccctccttggtcctccagttctaccactcagactccagtatgaaccgggctccaggatcccccgcgggttttctggatccaaagatgcctcagccaacgcagggctccttcttgtctctgggctgcagcctgagcacgaggctgactctgaccgtgcaggctggtgcaacagggcttct

SEQ ID NO: 170 - DNA, 246 bp, Bos taurus
  source 1..246: mol_type = genomic DNA
tgcaccctgcgcagtgacatcagtgtcggccactctgctcttactggaaccagcagaagccagcgagccctcctcggtcctctggtcctaccactgagactccagtaagaatcaggctccggggtcccccgtgggttttctggatccaaagatgcctcggccaatgtagggctcctgctcttctctgggctgcagcccgaggacgaggctgactctgaccgtgcaggctggtgcaacagggcttct

SEQ ID NO: 171 - DNA, 245 bp, Bos taurus; identical to SEQ ID NO: 167
  source 1..245: mol_type = genomic DNA

SEQ ID NO: 172 - DNA, 245 bp, Bos taurus
  source 1..245: mol_type = genomic DNA
tgcaccccgagcagtgacatcagtgtcagtcgctctgctgttactagaaccagcagaagccagcgagccctccttagtcctccggtcctaccactcagaccccagtaagaaccagtctttggggtccccgcgggttttctggatccaaagatgcctcagccaacgcggggctcctgctcgtctctgggctgcagcctgaggatgaggctgactctgaccatgcaggctggtgcaacagggcttct

SEQ ID NO: 173 - DNA, 206 bp, Bos taurus
  source 1..206: mol_type = genomic DNA
gttactggaaccagcagaagccagtgagccctcctccgccctccgatcctaccactcagactccagtaagaaccaggctccggggtcctcgcaggttttctggatccaaagatgcctcggccaatgcagggctcctgctcgtctccgggctgcagcctgaggatgaggctgactctgaccgtgcaggctggtgcaacagggcttct

SEQ ID NO: 174 - DNA, 198 bp, Bos taurus
  source 1..198: mol_type = genomic DNA
tgttactggaaccagcagaagccagcgagccctccttagtcctccggtcctaccactcagactccagtaagaaccagtcggggtccccgcgggttttctggatccaaagatgcctcagccaaggggctcctgctcgtctctgggctgcagcctgaggatgaggctactctaaccatgcaggctggtgcaacagggctt

SEQ ID NO: 175 - DNA, 206 bp, Bos taurus
  source 1..206: mol_type = genomic DNA
gttactggaaccagcagaagccagtgagcctcctccgccctccgatcctaccactcagactccagtacagaaccaggctccggggtcctcgcaggttttctggatccaaagatgcctcggccaatgcagggctcctgctcgtctccgggctgccacctgaggataggctggactctgaccgtgcaggctggtgcaacagggcttct

SEQ ID NO: 176 - DNA, 38 bp, Bos taurus
  source 1..38: mol_type = genomic DNA
ttttgtcttaggcggcgggacctgggtcaccgtcctgg

SEQ ID NO: 177 - DNA, 38 bp, Bos taurus
  source 1..38: mol_type = genomic DNA
tgatcttttcggcggcgggaccagagtgaccgtcctgg

SEQ ID NO: 178 - DNA, 38 bp, Bos taurus
  source 1..38: mol_type = genomic DNA
tgatcttttcggcggcgggaccacagtgaccgtcctgg

SEQ ID NO: 179 - DNA, 38 bp, Bos taurus
  source 1..38: mol_type = genomic DNA
tgctgttttcggcagcgggaccacactgaccgtcctgg

SEQ ID NO: 180 - DNA, 38 bp, Bos taurus
  source 1..38: mol_type = genomic DNA
tcctattttcattggcaggaccaggctgactgtcctgg

SEQ ID NO: 181 - DNA, 38 bp, Bos taurus; identical to SEQ ID NO: 179
  source 1..38: mol_type = genomic DNA

SEQ ID NO: 182 - DNA, 38 bp, Bos taurus; identical to SEQ ID NO: 179
  source 1..38: mol_type = genomic DNA

SEQ ID NO: 183 - DNA, 38 bp, Bos taurus; identical to SEQ ID NO: 180
  source 1..38: mol_type = genomic DNA

SEQ ID NO: 184 - DNA, 306 bp, Bos taurus
  modified_base 1: mod_base = OTHER; note = n = a, c, t, g, unknown or other
  source 1..306: mol_type = genomic DNA
nagagtgaaaccagccccagcatcttcccgctgagccttgggaacaacgacccagccgggcaggtggtcatcggctgcctggtccagggcttcttcccgtcggcacccctgagcgtgacctggaaccagaatggcgacagcgtgtccgtcaggaacttccctgccgtgctggccgggagcctgtacaccatgagcagccagctgaccttgccggccagcctgtgcccaaaaggccagtccgtgacctgccaagtgcagcacctctccaaagccagcaagaccgtggccgtgccctgcataattcaa

SEQ ID NO: 185 - DNA, 330 bp, Bos taurus
  source 1..330: mol_type = genomic DNA
gactcaagttcatgttgcgtgccgaactgcgagcccagcctgtccgtgcagccaccagccctcgaggacctgctcctgggctccaacgccagcctcacgtgcacactgagtggcctgaaaagcgccgagggcgccagcttcacctggaacccgacaggtgggaagaccgccgtccaggggtcgcccaagcgtgactcctgtggctgctacagcgtgtccagcgtcctgccgggctgtgccgatccctggaacagtggacagactttctcctgctctgtcacccaccccgagtccaagagttcactgaccgccaccatcaagaaagactta

SEQ ID NO: 186 - DNA, 393 bp, Bos taurus
  source 1..393: mol_type = genomic DNA
gggaacacgttccggcctcaggtccacctgctgccgccgccgtcggaggagctggccctcaacgagctggtgacgctgacgtgcctggtgcggggattcagccccaaggaggtgctggtgcgttggctgcagggcaatcaagagctgccccgcgagaagtatctgacctggggccccctgcccgaggctggccagagcgtcaccaccttcgccgtgaccagcgtgctacgcgtggacgccgaggtctggaagcagggggacaccttctcctgcatggtgggccacgaggccctgcccctggccttcacccagaagaccatcgaccgcctggcgggtaaacccacccacgtgaacgtgtccgtggtcatgtcagaggtggatggggtctgctac

SEQ ID NO: 187 - DNA, 186 bp, Bos taurus
  source 1..186: mol_type = genomic DNA
gaacatcagccctggctggtgctggacctgatgcagagcagccccgaggaggacagcccagaggccagcctgtggcccacgaccgtcaccctgctcaccctcttcctgctgagcctcttctacagcacagcactgactgtgacgagcatccggaccacgccggacagccgggaggtcccccagtac

SEQ ID NO: 188 - DNA, 324 bp, Bos taurus
  source 1..324: mol_type = genomic DNA
aaggtgaatcacacctgagagtcttccccctggtgtcctgcgtgagctccccatccgatgagagcacggtggccctgggctgcctggcccgggacttcgtgcccaattcagtcagcttctcctggaagttcaacaacagcacagtcagcagcgagagattctggaccttccccgaagtcctgagggacggcttgtggtcggcctcctctcaggtggtcctgccctcctcaagcgcctttcaagggccggatgactacctggtgtgtgaagtccagcaccccaagggaggaaagaccgtcggaaccgtgagggtggtccccagag

SEQ ID NO: 189 - DNA, 90 bp, Bos taurus
  source 1..90: mol_type = genomic DNA
catcgactccaaccccgaccactccattgccttctctgatatccgggtcagagggctccaacaaggcggtcagcacgcagagcagcccag

SEQ ID NO: 190 - DNA, 66 bp, Bos taurus
  source 1..66: mol_type = genomic DNA
cactgaccaccagccacagacagacagaagcccagacactggcgtgtccaaaggaaccctgcagag

SEQ ID NO: 191 - DNA, 324 bp, Bos taurus
  source 1..324: mol_type = genomic DNA
agtgtcagaaccacacccaggcccccagagtccacctgctgcccccaaccccccagggcctttggctcctggacaaggccgagttcacctgcctggccacgggggaggccccgctggatgcccacttctcctgggaggtgtacgggcagccccacggcggggccttggaggagggacccaccaggcacataaacagctcctggagccagagcagccgcctggccctgcccaggtccctgtgggcctcgggctccaacgtcacctgcacactgagcagccctggcctgcagtcgccggtgaccctgacggctcagagagaacatg

SEQ ID NO: 192 - DNA, 321 bp, Bos taurus
  source 1..321: mol_type = genomic DNA
ccgcctcagtgcctggcaatctgaccctccgcactgtgaccgcgcctggccccttctcccctgcctggctcctgtgcgaggtgtccggcttctcacccgtggacatcctcctcacgtggctggagagccagcaagaagtggagccttcccagtttgccacggcgcacaccacggcccaggctgggcgtgcctcatcccacacctggagtgtcctgcgtgtctccagccccctggaccacgcgggggccacctacacctgtgtggtcagccacgaggcctcccggacgctcctcaatggcagctgcagcctggacactggtg

SEQ ID NO: 193 - DNA, 147 bp, Bos taurus
  source 1..147: mol_type = genomic DNA
gtctggccacctggccaccggtggagcccaggacgagaagcagcgattgacggcacggatgtggaggatgccagcccactctggctcaccttcctggccctcttcctcgtcactgtggtctacggcggcttcgtcaccttcatcaag

SEQ ID NO: 194 - skipped

SEQ ID NO: 195 - DNA, 324 bp, Bos taurus
  source 1..324: mol_type = genomic DNA
aaggtgaatcgctcccgagagtcttccccttggtgtcctgcatgagctccccgtctgatgagagaatggtggccctgggctgcctggcccggatcttcatacccaattcgttcagcttctcctggaagttaaacaacagcacagtcagcagcgagagattctggaccttccccgcagtcctgagggacggcttgtggtcggcctcctctcaggtggccctgtcctcctcgagcgcctttcaagggccggatgactacctggtgtgtgaagtccagcaccccaagggaggaaagaccctcggccccgtgagggtgggccccagag

SEQ ID NO: 196 - DNA, 185 bp, Bos taurus
  source 1..185: mol_type = genomic DNA
ctcctgcctgtcattcacaggagctctcctgtgcgtctgagaagacctccctgacctccatggctgggccatggggcagctgggacccctggcctttacccgaacggagctcatccagggggtcctgtcatcgcatttagccgcctcaccggccccagaccactcacgcctgcattccatgtgtc

SEQ ID NO: 197 - DNA, 90 bp, Bos taurus; identical to SEQ ID NO: 189
  source 1..90: mol_type = genomic DNA

SEQ ID NO: 198 - DNA, 66 bp, Bos taurus
  source 1..66: mol_type = genomic DNA
cgccggccaccagccacagacagacagaagcccggacactggcatgtccaaaggacccctgcagag

SEQ ID NO: 199 - DNA, 325 bp, Bos taurus
  source 1..325: mol_type = genomic DNA
agtgtcagaaccacacccaggcccccagcgtccacctactgcccccaaaacccgcagggcctctggctcctggacaaggccgagttcacctgcctggccatgggggaggccccaccggatgtccacttctcctgggaggtgaacgggcagccccacggcgcggccttggaggagggacccacctggcacatgaacggctcctggagccagagcagccgcctggccctgcccaggtccctgtgggcctcaggctccaacgtcacctgcacactgagtggccccggcctgcggtcgccggtgaccctgatggctcagagagaacatg

SEQ ID NO: 200 - DNA, 321 bp, Bos taurus
  source 1..321: mol_type = genomic DNA
ccgcctcagtgcctggcaatctgaccctccgcactgtgaccgcgcctggccccttctcccctgcctggctcctgtgcgaggtgtccggcttctcacccgtggacatcctcctcacgtggctggagggccagcaagaagtggagccttcccagtttgccacggcacacaccacagcccaggctgggcacgcctcatcccacacctggagtgtcctgcgtgtctccagccccctggaccacgtgggggccacctacacctgtgtggtcagccacgaggcctcccggacgctcctcaatggcagctgcagcctggacactggtg

SEQ ID NO: 201 - DNA, 143 bp, Bos taurus
  source 1..143: mol_type = genomic DNA
gtctggccacctggccgccctggagccaggatgagagcagcgacgacggcacggatgtggaggatgccagcccactctggctcaccttcctggccctcgtcctcatcactgtggtctacggcggctttgtcaccttcatcaag

SEQ ID NO: 202 - skipped

SEQ ID NO: 203 - DNA, 100 bp, Bos taurus
  source 1..100: mol_type = genomic DNA
ttctcaagcacctttcaagggccggatgactacctggtgtgcgaagtccagcaccccaagggaggaaagaccgttggaaccgtgagggtggtccccagag

SEQ ID NO: 204 - DNA, 184 bp, Bos taurus
  source 1..184: mol_type = genomic DNA
ctcctgcctgtcattcacacgagctctcctgtgcgtctgagaagacctccctgactccatggctgggccatggggcagccgggacccctggcctttacccgaacggagctcatccagggggtcctgtcatcgcatttagccgcctcaccggccccagaccactcacccctgcattccatgtgtc

SEQ ID NO: 205 - DNA, 90 bp, Bos taurus
  source 1..90: mol_type = genomic DNA
catcgactccaaccccgaccacttcagtgccttctctgatatccgggtcagagggctccatcaaggccgtcagcacgcagagcagcccag

SEQ ID NO: 206 - DNA, 324 bp, Bos taurus
  source 1..324: mol_type = genomic DNA
agtgtcagaaccacacccaggcccccagcgtccacctgctgcccccaaccccccagggcctctggctcctggacaaggccgagttcacctgcctggccacgggggaggccccgctggatgcccgcttctcctgggaggtgaatgggcagccccacggcggggccttggaggagggacccacctggcacatgaacagctcctggagccagagcagccgcctggccctgcccaggtccctgtgggcctcaggctccaacgtcacctgcacactgagtggcccctgcctgcggtcaccggtgaccctgatggctcagagagaacatg

SEQ ID NO: 207 - DNA, 321 bp, Bos taurus
  source 1..321: mol_type = genomic DNA
ccgcctcagtgcccggcaatctgaccctccgcactgtgaccgcgcctggccccttctcccatgcctggctcctgtgcaaggtttccggcttctcacccgtggacatcctcctcacgtggctggagagccagcaagaagtggagccttcccagtttgccacggcgcacaccacggcccaggctgggcatgcctcatcccacacctggagtgtcctgcgtgtctccagccccctggaccacgcgggggccacctacacctgtgtggtcagccacgaggcctcccggacgctcctcaatggcagctgcagcctggacactggtg

SEQ ID NO: 208 - DNA, 143 bp, Bos taurus
  source 1..143: mol_type = genomic DNA
gtctggccacctggccaccgtggagccaggacgagagcagcgacgacggcacggatgtggaggatgccagcccactctggctcaccttcctggccctcttcctcgtcactgtggtctacggcggcttcgtcaccttcatcaag

SEQ ID NO: 209 - skipped

SEQ ID NO: 210 - DNA, 100 bp, Bos taurus; identical to SEQ ID NO: 203
  source 1..100: mol_type = genomic DNA

SEQ ID NO: 211 - DNA, 184 bp, Bos taurus; identical to SEQ ID NO: 204
  source 1..184: mol_type = genomic DNA

SEQ ID NO: 212 - DNA, 90 bp, Bos taurus; identical to SEQ ID NO: 205
  source 1..90: mol_type = genomic DNA

SEQ ID NO: 213 - DNA, 324 bp, Bos taurus
  source 1..324: mol_type = genomic DNA
agtgtcagaaccacacccaggcccccagcgtccacctgctgcccccaaccccccagggcctctggctcctggacaaggccgagttcacctgcctggccacgggggaggccccgctggatgcccgcttctcctgggaggtaaatgggcagccccacggcggggccttggaggagggacccacctggcacatgaacagctcctggagccagagcagccgcctggccctgcccaggtccctgtgggcctcaggctccaacgtcacctgcacactgagtggcccctgcctgcggtcaccggtgaccctgatggctcagagagaacatg

SEQ ID NO: 214 - DNA, 321 bp, Bos taurus
  source 1..321: mol_type = genomic DNA
ccgcctcagtgcccggcaatctgaccctccgcactgtgaccgtgcctggccccttctcccatgcctggctcctgtgcgaggtgtccggcttctcacccgtggacatcctcctcacgtggctggagagccagcaagaagtggagccttcccagtttgccacggcgcacaccacggcccaggctgggcgtgcctcatcccacacctggagtgtcctgcgtgtctccagccccctggaccacgcgggggccacctacacctgtgtggtcagccacgaggcctcccggacgctcctcaatggcagctgcagcctggacactggtg

SEQ ID NO: 215 - DNA, 143 bp, Bos taurus; identical to SEQ ID NO: 208
  source 1..143: mol_type = genomic DNA

SEQ ID NO: 216 - skipped

SEQ ID NO: 217 - DNA, 291 bp, Bos taurus
  modified_base 1: mod_base = OTHER; note = n = a, c, t, g, unknown or other
  source 1..291: mol_type = genomic DNA
ncctccatccaggctccatccatctaccccttgaggctctgttgcacagaagaagcccgtgtaaggctgggctgcctggtcaaggactacttgccagggtcagtgactgtgacctgggacacagtgcccctggatggaagcaccctgaccttccctagcatccaaatggcgagctccagtctctacattaccaccagccagctgaccatctcgggcgagcagcccaaggagttcacctgcagagttttacacgctgagaccaactccaacttgaataagaccatcagcact

SEQ ID NO: 218 - DNA, 324 bp, Bos taurus
  source 1..324: mol_type = genomic DNA
gagtgcgccaagaacttcagcgacccctcagtgaagctcttctactcctcctgcaaccccaatggcgacacccagaccaccatccacctcctgtgccggatctccggctacaccccgggcaaaatcaaggtcacctggctggtggatgggctcaagtccgaagagctgtatgcacgatccggccctgagatacaggagggcaatctgacctccacctacagtgaagtcaacatcacacagggccagtgggtgtccgagaaaacctacacctgccgggtcaactattacggctacaacttcgaaagccacgcccacaggtgcaca

SEQ ID NO: 219 - DNA, 324 bp, Bos taurus
  source 1..324: mol_type = genomic DNA
gccgagtccgagccccgcggcgtgagcgcctacctgagcccacccacccccctcgagctgtacgtcaacaagtcacccaagatcacctgcctggttgtggacctggccaacgagaagaacttgagcctgacctggtcgagggcaaacgggaagcctgtgcacgcaggcccccctgagatcaagcgtcagttcaacgggacggtcaccgtcacgtccaccctgccggtggacgtcactgactgggtagaaggcgagacctactactgcaaagtgagccacagcgacctgcccacggacatccagcgatccatctccaaggatgtt

SEQ ID NO: 220 - DNA, 339 bp, Bos taurus
  source 1..339: mol_type = genomic DNA
ggcaagcgtctggcccccaaggcctacgtgttcttgccagacggaaaggagctggagaacgaggaggagctcaccctcacctgcatgatccagaaattcttccccagggacatctttgtgcggtggctgcataacaaggaactgatgcgggcagaccagcacaccaccacacagccccacagggccgacaacaacaccccagccttcttcgcctacagccgcctggcggtccctagggccaactggaagaggggcgatgagttcacctgccaagtgatccatgaggcactgcccaggactaggaccctggagaaatcggtgttcattaacagcggtaaa

SEQ ID NO: 221 - DNA, 135 bp, Bos taurus
  source 1..135: mol_type = genomic DNA
gagctggccctcgaggacctgtgtgcagaggaagctgagagcgaggagctggaggagacctggaccagcctccttgtcttcatcgtgctcttcctgctcagcatgagctatggcgccgccgtcagcctctgcaag

SEQ ID NO: 222 - DNA, 93 bp, Bos taurus
  source 1..93: mol_type = genomic DNA
gtgaagtggatcctggccgccatcctccaggggcagccccagggctcccaagactacaccaacgtcacacagcgcccactgcctgctggtgtc

SEQ ID NO: 223 - DNA, 291 bp, Bos taurus
  modified_base 1: mod_base = OTHER; note = n = a, c, t, g, unknown or other
  source 1..291: mol_type = genomic DNA
ncctccaccacagccccgaaagtctaccctctgagttcttgctgcggggacaagtccagctccaccgtgaccctgggctgcctggtctccagctacatgcccgagccggtgaccgtgacctggaactcgggtgccctgaagagcggcgtgcacaccttcccggctgtccttcagtcctccgggctctactctctcagcagcatggtgaccgtgcccggcagcagctcaggacagaccttcacctgcaacgtagcccacccggccagcagcaccaaggtggacaaggctgtt

SEQ ID NO: 224 - DNA, 36 bp, Bos taurus
  source 1..36: mol_type = genomic DNA
gatcccagatgcaaaacaacctgtgactgttgccca

SEQ ID NO: 225 - DNA, 330 bp, Bos taurus
  source 1..330: mol_type = genomic DNA
ccgcctgagctccctggaggaccctctgtcttcatcttcccaccgaaacccaaggacaccctcacaatctcgggaacgcccgaggtcacgtgtgtggtggtggacgtgggccacgatgaccccgaggtgaagttctcctggttcgtggacgacgtggaggtaaacacagccacgacgaagccgagagaggagcagttcaacagcacctaccgcgtggtcagcgccctgcgcatccagcaccaggactggactggaggaaaggagttcaagtgcaaggtccacaacgaaggcctcccggcccccatcgtgaggaccatctccaggaccaaa

SEQ ID NO: 226 - DNA, 327 bp, Bos taurus
  source 1..327: mol_type = genomic DNA
gggccggcccgggagccgcaggtgtatgtcctggccccaccccaggaagagctcagcaaaagcacggtcagcctcacctgcatggtcaccagcttctacccagactacatcgccgtggagtggcagagaaatgggcagcctgagtcagaggacaagtacggcacgacccctccccagctggacgccgacggctcctacttcctgtacagcaggctcagggtggacaggaacagctggcaggaaggagacacctacacgtgtgtggtgatgcacgaggccctgcacaatcactacacgcagaagtccacctctaagtctgcgggtaaa

SEQ ID NO: 227 - DNA, 135 bp, Bos taurus
  source 1..135: mol_type = genomic DNA
gacctgctgctggaggaggagatctgtgcggacgcccaggacggggagctggacgggctctggacgactatctccatcttcatcacactcttcctgctcagcgtctgctacagcgccaccgtgaccctcttcaag

SEQ ID NO: 228 - DNA, 81 bp, Bos taurus
  source 1..81: mol_type = genomic DNA
gtgaagtggatcttctcatcagtggtggagctgaagaggacgatcgtccccgactacagaaatatgatcgggcagggagcc

SEQ ID NO: 229 - DNA, 291 bp, Bos taurus
  modified_base 1: mod_base = OTHER; note = n = a, c, t, g, unknown or other
  source 1..291: mol_type = genomic DNA
ncctccaccacagccccgaaagtctaccctctggcatcccgctgcggagacacatccagctccaccgtgaccctgggctgcctggtctccagctacatgcccgagccggtgaccgtgacctggaactcgggtgccctgaagagcggcgtgcacaccttcccggccgtccttcagtcctccgggctctactctctcagcagcatggtgaccgtgcccggcagcagctcaggacagaccttcacctgcaacgtagcccacccggccagcagcaccaaggtggacaaggctgtt

SEQ ID NO: 230 - DNA, 39 bp, Bos taurus
  source 1..39: mol_type = genomic DNA
ggggtctccattgactgctccaagtgtcataaccagcct

SEQ ID NO: 231 - DNA, 321 bp, Bos taurus
  source 1..321: mol_type = genomic DNA
tgcgtgagggaaccatctgtcttcatcttcccaccgaaacccaaagacaccctgatgatcacaggaacgcccgaggtcacgtgtgtggtggtgaacgtgggccacgataaccccgaggtgcagttctcctggttcgtggatgacgtggaggtgcacacggccaggtcgaagccaagagaggagcagttcaacagcacgtaccgcgtggtcagcgccctgcccatccagcaccaggactggactggaggaaaggagttcaagtgcaaggtcaacaacaaaggcctctcggcccccatcgtgaggatcatctccaggagcaaa

SEQ ID NO: 232 - DNA, 327 bp, Bos taurus
  source 1..327: mol_type = genomic DNA
gggccggcccgggagccgcaggtgtatgtcctggacccacccaaggaagagctcagcaaaagcacgctcagcgtcacctgcatggtcaccggcttctacccagaagatgtagccgtggagtggcagagaaaccggcagactgagtcggaggacaagtaccgcacgaccccgccccagctggacaccgaccgctcctacttcctgtacagcaagctcagggtggacaggaacagctggcaggaaggagacacctacacgtgtgtggtgatgcacgaggccctgcacaatcactacatgcagaagtccacctctaagtctgcgggtaaa

SEQ ID NO: 233 - DNA, 135 bp, Bos taurus
  source 1..135: mol_type = genomic DNA
gacctgctgctggaggaggagatctgtgcggacgcccaggacggggagctggacgggctctggacgactatctccatcttcatcacactctttctgctcagcgtctgctacagcgccaccgtgaccctcttcaag

SEQ ID NO: 234 - DNA, 81 bp, Bos taurus
  source 1..81: mol_type = genomic DNA
gtgaagtggatcctctcatccgtggtggagctgaagcagtcgatcactcccaactacagaaacatgatcggacagggcgcc

SEQ ID NO: 235 - DNA, 294 bp, Bos taurus
  modified_base 1: mod_base = OTHER; note = n = a, c, t, g, unknown or other
  source 1..294: mol_type = genomic DNA
ncctccaccacagccccgaaagtctaccctctggcatccagctgcggagacacatccagctccaccgtgaccctgggctgcctggtctccagctacatgcccgagccggtgaccgtgacctggaactcgggtgccctgaagagcggcgtgcacaccttcccggccgtccggcagtcctctgggctgtactctctcagcagcatggtgaccgtgcccgccagcacctcaggaacccagaccttcacctgcaacgtagcccacccggccagcagcaccaaggtggacaaggctgtc

SEQ ID NO: 236 - DNA, 66 bp, Bos taurus
  source 1..66: mol_type = genomic DNA
actgcaaggcgtccagtcccgacgacgccaaagacaaccatccctcctggaaaacccacaacccag

SEQ ID NO: 237 - DNA, 45 bp, Bos taurus
  source 1..45: mol_type = genomic DNA
gagcctgaagttgaaaagacaccctgccagtgttccaaatgccca

SEQ ID NO: 238 - DNA, 324 bp, Bos taurus
  source 1..324: mol_type = genomic DNA
gaacctccgggaggactgtctgtcttcatcttcccaccgaaacccaaggacaccctcacaatctcaggaacgcccgaggtcacgtgtgtggtggtggacgtgggccaggatgaccccgaggtgcagttctcctggttcgtggacgacgtggaggtgcacacggccaggacgaagccgagagaggagcagttcaacagcacctaccgcgtggtcagcgccctgcgcatccagcaccaggactggctgcagggaaaggagttcaagtgcaaggtcaacaacaaaggcctcccggcccccattgtgaggaccatctccaggaccaaa

SEQ ID NO: 239 - DNA, 327 bp, Bos taurus
  source 1..327: mol_type = genomic DNA
gggcaggcccgggagccgctggtgtatgtcctggccccaccccgggaagagctcagcaaaagcacgctcagcctcacctgcctgatcaccggtttctacccagaagagatagacgtggagtggcagagaaatgggcagcctgagtcagaggacaagtaccacacgaccgcaccccagctggatgctgacggctcctacttcctgtacagcaggctcagggtgaacaagagcagctggcaggaaggagaccactacacgtgtgcagtgatgcatgaagctttacggaatcactacaaagagaagtccatctcgaggtctccgggtaaa

SEQ ID NO: 240 - DNA, 135 bp, Bos taurus
  source 1..135: mol_type = genomic DNA
gacttgctgctggaggaggagatctgtgcggacgacctggatggggagctggacgggctctggacgactatctccatcttcatcacactcttcctgctcagcgtctgctacagcgccactgtgaccctcttcaag

SEQ ID NO: 241 - DNA, 81 bp, Bos taurus
  source 1..81: mol_type = genomic DNA
gtgaaatggatcttctcctcggcggtggagctgaagaggacgatcgtccccgactacagaaacatgctcgggcagggcgcc

SEQ ID NO: 242 - DNA, 294 bp, Bos taurus; identical to SEQ ID NO: 235
  modified_base 1: mod_base = OTHER; note = n = a, c, t, g, unknown or other
  source 1..294: mol_type = genomic DNA

SEQ ID NO: 243 - DNA, 66 bp, Bos taurus; identical to SEQ ID NO: 236
  source 1..66: mol_type = genomic DNA

SEQ ID NO: 244 - DNA, 45 bp, Bos taurus; identical to SEQ ID NO: 237
  source 1..45: mol_type = genomic DNA

SEQ ID NO: 245 - DNA, 324 bp, Bos taurus; identical to SEQ ID NO: 238
  source 1..324: mol_type = genomic DNA

SEQ ID NO: 246 - DNA, 327 bp, Bos taurus; identical to SEQ ID NO: 239
  source 1..327: mol_type = genomic DNA

SEQ ID NO: 247 - DNA, 135 bp, Bos taurus; identical to SEQ ID NO: 240
  source 1..135: mol_type = genomic DNA

SEQ ID NO: 248 - DNA, 81 bp, Bos taurus; identical to SEQ ID NO: 241
  source 1..81: mol_type = genomic DNA

SEQ ID NO: 249 - DNA, 288 bp, Bos taurus
  source 1..288: mol_type = genomic DNA
cctccaccacagccccgaaagtctaccctctggcatccagctgcggagacacatccagctccaccgtgaccctgggctgcctggtctccagctacatgcccgagccggtgaccgtgacctggaactcgggtgccctgaagagcggcgtgcacaccttcccggccgtccggcagtcctctgggctgtactctctcagcagcatggtgaccgtgcccgccagcagctcagaaacccagaccttcacctgcaacgtagcccacccggccagcagcaccaaggtggacaagg

SEQ ID NO: 250 - DNA, 45 bp, Bos taurus
  source 1..45: mol_type = genomic DNA
agtctgaagttgaaaagacaccctgccagtgttccaaatgcccag

SEQ ID NO: 251 - DNA, 324 bp, Bos taurus
  source 1..324: mol_type = genomic DNA
aacctctgggaggactgtctgtcttcatcttcccaccgaaacccaaggacaacctacacatctcgggaacgcccgaggttacgtgtgtggtggtggacgtgggccaggatgaccccgaggtgcagttctcctggttcgtggacgacgtggaggtgcacacggccaggacgaagccgagagaggagcagttcaacagcacctaccgcgtggtcagcgccctgcgcatccagcaccaggactggctgcagggaaaggagttcaagtgcaaggtcaacaacaaaggcctcccggcccccattgtgaggaccatctccaggaccaaag

SEQ ID NO: 252 - DNA, 325 bp, Bos taurus
  source 1..325: mol_type = genomic DNA
ggcaggcccgggagccgcaggtgtatgtcctggccccacccgggaagagctcagcaaaagcacgctcagcctcacctgcctgatcaccggtttctacccagaagagatagacgtggagtggcagagaaatgggcagcctgagtcggaggacaagtaccacacgaccgcaccccagctggatgctgacggctcctacttcctgtacagcaggctcagggtgaacaagagcagctggcaggaaggagaccactacacgtgtgcagtgatgcatgaagctttacggaatcactacaaagagaagtccatctcgaggtctccgggtaaa

SEQ ID NO: 253 - DNA, 324 bp, Bos taurus
  modified_base 1: mod_base = OTHER; note = n = a, c, t, g, unknown or other
  source 1..324: mol_type = genomic DNA
naaggtgaatcacacccgaaagtcttccccctggtgtcctgcgtgagctcgccatccgatgagagcacggtggccctgggctgcctggcccgggacttcgtgcccaattcagtcagcttctcctggaagttcaacaacagcacagtcagcagcgagagattctggaccttccccgaagtcctgagggacggcttgtggtcggcctcctctcaggtggtcctgccctcctcaagcgcctttcaagggccggatgactacctggtgtgcgaagtccagcaccccaagggaggaaagaccgtcggcaccgtgagggtgatcgctaca

SEQ ID NO: 254 - DNA, 333 bp, Bos taurus
  source 1..333: mol_type = genomic DNA
aaggcggaagtgctgtccccagtcgtgagtgtctttgtcccgcctcgcaacagcctctctggtgacggcaatagcaagtccagcctcatctgccaggccacggacttcagccccaaacagatctcgttgtcctggtttcgtgatggaaagcggatagtgtctggaatttctgaaggccaggtggagactgtgcagtcctcacccataaccttcagggcctacagcatgctgaccatcacggagagagactggctcagccagaacgcgtacacctgccaggtagaacacaacaaggaaaccttccagaagaacgtgtcctcctcatgtgatgtt

SEQ ID NO: 255 - DNA, 315 bp, Bos taurus
  source 1..315: mol_type = genomic DNA
gcaccaccatctccgatcggggtcttcaccatccccccatccttcgccgacatcttcctcacgaagtcagccaagctgtcctgtctggtcacaaacctggcctcctatgatggcctgaacatcagctggtcccgtcagaacgccaaggccctggagacccacacgtattttgagcgacacctcaacgacaccttcagcgcccggggtgaggcctcggtctgctcggaggactgggagtccggagaggagttcacgtgcacagtggcccactcggacctgcccttcccagaaaagaacgccgtctccaagcccaaa

SEQ ID NO: 256 - DNA, 393 bp, Bos taurus
  source 1..393: mol_type = genomic DNA
gacgtcgccatgaaaccgccgtccgtgtacctgctgcctccaacgcgggaacagctgagcctgcgcgagtcggcctccgtcacctgcctggtgaaggcgttcgcgcccgcggacgtgttcgtgcagtggctgcagaggggggagcccgtgaccaagagcaagtacgtgaccagcgcccgcgcgcccgagccccaggaccccagcgtggtgtactttgtgcacagcatcctgacggtggccgaggaggactggagcaaaggggagacctacacctgcgtcgtgcacgaagccctgccccacatggtcaccgagcggaccgtggacaagtccaccggtaaacccaccctgtacaacgtgtccctggtcctgtctgacacagccagcacctgctac

SEQ ID NO: 257 - DNA, 117 bp, Bos taurus
  source 1..117: mol_type = genomic DNA
gagggggaggtgagcgccgaggaagaaggctttgaaaacctcaacaccatggcctccaccttcatcgtgctcttcctcctgagcctcttctacagcaccacggtcaccctgttcaag

SEQ ID NO: 258 - skipped

SEQ ID NO: 259 - DNA, 324 bp, Bos taurus
  modified_base 1: mod_base = OTHER; note = n = a, c, t, g, unknown or other
  source 1..324: mol_type = genomic DNA
naaggtgaatcacacccgagagtcttccccctggtgtcctgcgtgagctccccatccgatgagagcacggtggccctgggctgcctggcccgggacttcgtgcccaattcagtcagcttctcctggaagttcaacaacagcacagtcagcagcgagagattctggaccttccccgaagtcctgagggacggcttgtggtcggcctcctctcaggtggtcctgccctcctcaagcgcctttcaagggccggatgactacctggtgtgcgaagtccagcaccccaagggaggaaagaccgtcggcaccgtgagggtggtcgctaca

SEQ ID NO: 260 - DNA, 333 bp, Bos taurus
  source 1..333: mol_type = genomic DNA
aaggcggaagtgctgtccccagtcgtgagtgtctttgtcccgcctcgcaacagcctctctggtgacggcaatagcaagtccagcctcatctgccaggccacggacttcagccccaaacagatctccttgtcctggtttcgtgatggaaagcggatagtgtctggcatttctgaaggccaggtggagactgtgcagtcctcacccgtaactttcagggcctacagcatgctgaccatcacggagagagactggctcagccagaacgtgtacacctgccaggtagaacacaacaaggaaaccttccagaagaacgtgtcctcctcatgtgatgtt

SEQ ID NO: 261 - DNA, 315 bp, Bos taurus
  source 1..315: mol_type = genomic DNA
gcaccaccatctcccatcggggtcttcaccatccccccatccttcgccgacatcttcctcacgaagtcagccaagctgtcctgtctggtcacaaacctggcctcctatgatggcctgaacatcagctggtcccgtcagaacggcaaggccctggagacccacacgtattttgagcgacacctcaacgacaccttcagcgcccggggtgaggcctcggtctgctcggaggactgggagtccggagaggagttcacgtgcacagtggcccactcggacctgcccttcccagaaaagaacaccgtctccaagcccaaa

SEQ ID NO: 262 - DNA, 393 bp, Bos taurus
  source 1..393: mol_type = genomic DNA
gatgtcgccatgaaaccgccgtccgtgtacctgctgcctccaacgcgggaacagctgagcctgcgggagtcggcctccgtcacctgcctggtgaagggcttcgcgcccgcggacgtgttcgtgcagtggctgcagaggggggagcccgtgaccaagagcaagtacgtgaccagcagcccggcgcccgagccccaggaccccagcgtgtactttgtgcacagcatcctgacggtggccgaggaggactggagcaaaggggagacctacacctgcgtcgtgggccacgaggccctgccccacatggtcaccgagcggaccgtggacaagtccaccggtaaacccaccctgtacaacgtgtccctggtcctgtctgacacagccagcacctgctac

SEQ ID NO: 263 - DNA, 117 bp, Bos taurus
  source 1..117: mol_type = genomic DNA
gagggggaggtgagcgccgaggaggaaggctttgagaacctcaacaccatggcctccaccttcatcgtgctcttcctcctgagcctcttctacagcaccacggtcaccctgttcaag

SEQ ID NO: 264 - skipped

SEQ ID NO: 265 - DNA, 324 bp, Bos taurus
  modified_base 1: mod_base = OTHER; note = n = a, c, t, g, unknown or other
  source 1..324: mol_type = other DNA
nggtctgatgctgagccatccgtcttcctcttcaaaccatctgatgagcagctgaagaccggaactgtctctgtcgtgtgcttggtgaatgatttctaccccaaagatatcaatgtcaagtggaaagtggatggggttactcagagcagcagcaacttccaaaacagtttcacagaccaggacagcaagaaaagcacctacagcctcagcagcatcctgacactgcccagctcagagtaccaaagccatgacgcctatacgtgtgaggtcagccacaagagcctgactaccaccctcgtcaagagcttcagtaagaacgagtgt

SEQ ID NO: 266 - DNA, 316 bp, Bos taurus
  source 1..316: mol_type = genomic DNA
gtcagcccaagtccgcaccctcggtcaccctgttcccgccccccaccgaggagctcagcgccaacaaggccaccctggtgtgtctcatcagtgacttctacccgggtagcgtgaccgtggcctggaaggcagacggcagcaccatcacccgcaacgtggagaccacccgggcctccaaacagagcaacagcaagtacgcggccagcagctactgagcctgacgggcagcgactggaaatcgaaaggcagttacagctgcgaggtcacgcacgaggggagcaccgtgacgaagacagtgaagacctcagcgtgttct

SEQ ID NO: 267 - DNA, 318 bp, Bos taurus
  source 1..318: mol_type = genomic DNA
ggtcagcccaagtccccaccctcggtcaccctgttcccgccctccaaggaggagctcagcgccaacaaggccaccctggtgtgtctcatcagcgacttctacccgggtagcgtgaccgtggcctggaaggcagacggcagcaccatcacccgcaacgtgaagaccacccgggcctccaaacagagcaacagcaagtacgcggccagcagctacctgagcctgacagacagcgactggaaatcgaaaggcagttacagctgcgaggtcacgcacgaggggagcaccgtgacgaagacagtgaagacctcagcgtgttct

SEQ ID NO: 268 - DNA, 318 bp, Bos taurus
  source 1..318: mol_type = genomic DNA
ggtcagcccaagtccccaccctcggtcaccctgttcccgccctccaaggaggagctcagcgccaacaaggccaccctggtgtgtctcatcagcgacttctacccgggtagcgtgaccgtggcctggaaggcagacggcagcaccatcacccgcaacgtggagaccacccgggcctccaaacagagcaacagcaagtacgcggccagcagctacctgagcctgacgagcagcgactggaaatcgaaaggcagttacagctgcgaggtcacgcacgaggggagcaccgtgacgaagacagtgaagacctcagcgtgttct

SEQ ID NO: 269 - DNA, 318 bp, Bos taurus
  source 1..318: mol_type = genomic DNA
ggtcagcccaagtccccaccctcggtcaccctgttcccgccctccacggaggagctcaacggcaacaaggccaccctggtgtgtctcatcagcgacttctacccgggtagcgtgaccgtggtctggaaggcagacggcagcaccatcacccgcaacgtggagaccacccgggcctccaaacagagcaacagcaagtacgcggccagcagctacctgagcctgacgagcagcgactggaaatcgaaaggcagttacagctgcgaggtcacgcacgaggggagcaccgtgacgaagacagtgaagccctcagagtgttct

SEQ ID NO: 270 - DNA, 315 bp, Bos taurus
  source 1..315: mol_type = genomic DNA
gtcagcccaagtccacacctcggtcaccctgttcccgccctccaaggaggagctcagcaccaacaaggccaccctggtgtgtctcatcagcgacttctacccgggtagcgtgaccgtggtctagaaggcagacggcagcaccatcacccacaacgtggagaccacccgggcctccaaacagagcaacagcaagtaccgcggccagcagctacctgagcctgatgggcagcgactggaaatcgaaaggcagttacagctgcgaggtcacgcacgagggagcaccgtgacgaagacagtgaagcctcagagtgttct

SEQ ID NO: 271 - DNA, 314 bp, Bos taurus
  source 1..314: mol_type = genomic DNA
gtcagcccaagttcacaccctcgtcactgtttccgcccacctccaaggagagccagcaccaacaaggccaacccctgtgtgtctcatcagcgacttctaccccggtagtcgtacccgggtcagaaggcagaacggcaaccatctacccacaacgtggagaccacccggccccaaacagagcaccagcaagtaacgcggccgagcactacccacctgagcctgatggcagcgacggaaaatcgaaaggctagttacagcgcgagttcagcacgaaggggagcacgtgacgaaacatgaagcctcagagtgttcct

SEQ ID NO: 272 - DNA, 316 bp, Bos taurus
  source 1..316: mol_type = genomic DNA
gtcagcccaagtccccaccctcgtcaccctgttcccgccctccacggaggagctcaacggcaacaaggccaccctggtgtgtctcatcagcgacttctacccgggtagcgtgaccgtggtctggaaggcagacggcagcaccatcacccgcaacgtggagaccacccgggcctccaaacagagcaacagcaagtacgcggccagcagctacctgagcctgacgagcagcgactggaaatcgaaaggcagttacagctgcgaggtcacgcacgaggggagcaccgtgacgaagacagtgaagccctcagagtgttct

SEQ ID NO: 273 - DNA, 318 bp, Bos taurus; identical to SEQ ID NO: 269
  source 1..318: mol_type = genomic DNA

SEQ ID NO: 274 - DNA, 316 bp, Bos taurus
  source 1..316: mol_type = genomic DNA
gtcagcccaagtccacaccctcggtcaccctgttcccgccctccaaggaggagctcagcaccaacaaggccaccctggtgtgtctcatcagcgacttctacccgggtagcgtgaccgtggtctagaaggcagacggcagcaccatcacccacaacgtggagaccacccgggcctccaaacagagcaacagcaagtacgcggccagcagctacctgagcctgatgggcagcgactggaaatcgaaaggcagttacagctgcgaggtcacgcacgaggggagcaccgtgacgaagacagtgaagcctcagagtgttct

SEQ ID NO: 275 - DNA, 24 bp, synthetic construct
  misc_feature 1..24: note = source = /note="Description of Artificial Sequence: Synthetic primer"
  source 1..24: mol_type = other DNA
acataatacactgaaatggagccc

SEQ ID NO: 276 - DNA, 20 bp, synthetic construct
  misc_feature 1..20: note = source = /note="Description of Artificial Sequence: Synthetic primer"
  source 1..20: mol_type = other DNA
gtccttggtcaacgtgaggg

SEQ ID NO: 277 - DNA, 24 bp, synthetic construct
  misc_feature 1..24: note = source = /note="Description of Artificial Sequence: Synthetic primer"
  source 1..24: mol_type = other DNA
cataatacactgaaatggagccct

SEQ ID NO: 278 - DNA, 20 bp, synthetic construct
  misc_feature 1..20: note = source = /note="Description of Artificial Sequence: Synthetic primer"
  source 1..20: mol_type = other DNA
gcaacagtggtaggtcgctt

SEQ ID NO: 279 - DNA, 100 bp, Mus musculus
  source 1..100: mol_type = genomic DNA
atttctgtacctgatctatgtcaatatctgtaccatggctctagcagagatgaaatatgagacagtctgatgtcatgtggccatgcctggtccagacttg

SEQ ID NO: 280 - DNA, 100 bp, Mus musculus
  source 1..100: mol_type = genomic DNA
gtcaatcagcagaaatccatcatacatgagacaaagttataatcaagaaatgttgcccataggaaacagaggatatctctagcactcagagactgagcac

SEQ ID NO: 281 - DNA, 1103 bp, Mus musculus
  source 1..1103: mol_type = genomic DNA
gcattgaataaaccagtataaacaagcaagcaaagatagatagatagatagatagatagatagatagatacatagatagatagatagatagatagatgatagatagatagatagatagatagatttttacgtataatacaataaaaacattcattgtccctctattggtgactactcaaggaaaaaaatgttcatatgcaagaaaaaatgttatcattaccagatgatccagcaatctagcaatatatatattgtttattcacaaaacatgaatgaaccttttaagaagctgttacagtgtaaaaattaagttaaatcactgaagaacatatactgtgtgatttcattcaaatgaaatttgagaagtaaatatatatgtatatatatatatatgtaaaaaatataagtctgaactacaaaaattcaatttgtttgatatgtaagaataagaaaaattgacccccaaaatttgttaataattaggtatgtgtatttttatgaatatataagtataataatgcttatagtatacactattctgaatcacatttattccctaagtgtgttcccttgattataattaaaagtatattttttaaatacagagtcagagtacagtcaataaggcgaaaatatagttgaatgatttgcttcagcttttgtaatgtactagagattgtgagtacaaagtctcagagctcattttatccctgacaataaccagctctgtgcttcaagtacatttccatctttctctgaaatttagtcttatatagatagacaaaatttaagtaaatttcaaactacacagaacaactaagttgttgtttcatattgataatggatttgaactgcattaacagaactttaacatcctgcttattctcccttcagccatcatattttgctttattattttcactttttgagttatttttcacattcagaaagctcacataattgtcacttctttgtatactggtatacagaccagaacatttgcatattgttccctggggaggtctttgccctgttggcctgagataaaacctcaagtgtcctcttgcctccactgatcactctcctatgtttatttcctcaaa

SEQ ID NO: 282 - DNA, 49 bp, cow
  source 1..49: mol_type = genomic DNA
atgagattctctgctcagctcctggggctcctcctgctctgggtcccag

SEQ ID NO: 283 - DNA, 401 bp, cow
  source 1..401: mol_type = genomic DNA
gtaagtacagagagggatgagaaggaggatgggggtgagttctggggcagcactgctctccacatgtgttctctgttagatgtgtatgacttgtcctgcagatgagcatgggaaccttagatcaatgatagtgaggaatgttccagaaggaagaaggtcctgtgctctggtcaggactgtgacaggggaagtggggatgatgtaggggatgtttagaggtctctttatacttcacagatatcaagttcattattgtgattgtacaattttgctgtatgatcacagacaatgtgagtaatacaaagtagtattaatgttttagctaaaataaatcagaaaatggaaacaataaaaatggttgctaatatttgtagctttctaattctctgtcattcctttag

SEQ ID NO: 284 - DNA, 308 bp, cow
  source 1..308: mol_type = genomic DNA
gatccagtggggatgttgtgctgacccagactccactctccctgtctatcatccctggagagatggcctccatctcctgcaagtctagtcagagcctggtacacagtgatggaaaaacctatttgaattggattcaatataaaccaggccaatcaccacagggtctgatctatcaggtttccaaccgttactctggggtctcagacaggttcactggcagtgggtcagggacagatttcacacttacaatcagcagagtgcaggctgaggatgctggagtctattactgttaccaaggtacagaagat

SEQ ID NO: 285 - skipped

SEQ ID NO: 286 - DNA, 142 bp, Mus musculus
  source 1..142: mol_type = genomic DNA
atacagactctatcaaaaacttccttgcctggggcagcccagctgacaatgtgcaatctgaagaggagcagagagcatcttgtgtctgtgtgagaaggaggggctgggatacatgagtaattctttgcagctgtgagctctg

SEQ ID NO: 287 - DNA, 1103 bp, Mus musculus; identical to SEQ ID NO: 281
  source 1..1103: mol_type = genomic DNA

SEQ ID NO: 288 - DNA, 49 bp, Mus musculus
  source 1..49: mol_type = genomic DNA
atgatgagtcctgcccagttcctgtttctgttagtgctctggattcagg

SEQ ID NO: 289 - DNA, 386 bp, Mus musculus
  source 1..386: mol_type = genomic DNA
gtaaggagttttggaatgtgagggatgagaatggggatggagggtgatctctggatgcctatgtgtgctgtttatttgtggtggggcaggtcatatcttccagaatgtgaggttttgttacatcctaatgagatattccacatggaacagtatctgtactaagatcagtattctgacatagattggatggagtggtatagactccatctataatggatgatgtttagaaacttcaacacttgttttatgacaaagcatttgatatataatatttttaaatctgaaaaactgctaggatcttacttgaaaggaatagcataaaagatttcacaaaggttgctcaggatctttgcacatgattttccactattgtattgtaatttcag

SEQ ID NO: 290 - DNA, 11 bp, Mus musculus
  source 1..11: mol_type = genomic DNA
aaaccaacggt

SEQ ID NO: 291 - DNA, 308 bp, cow; identical to SEQ ID NO: 284
  source 1..308: mol_type = genomic DNA

SEQ ID NO: 292 - skipped

SEQ ID NO: 293 - DNA, 142 bp, Mus musculus; identical to SEQ ID NO: 286
  source 1..142: mol_type = genomic DNA

SEQ ID NO: 294 - DNA, 13 bp, Mus musculus
  source 1..13: mol_type = genomic DNA
cttccttcctcag

SEQ ID NO: 295 - DNA, 13 bp, synthetic construct
  misc_feature 1..13: note = source = /note="Description of Artificial Sequence: Synthetic oligonucleotide"
  source 1..13: mol_type = other DNA
aaattaattaacc